European Patent Application EP 4 653 056 A2, published November 26, 2025. Title: HUMAN ANTIBODIES TO FEL D1 AND METHODS OF USE THEREOF. Applicant: REGENERON PHARMACEUTICALS, INC. Application EP. The sequence listing filed with the application follows.

SEQUENCE LISTING (490 sequences)

SEQ ID NO: 1 - DNA, 363 bp, synthetic construct
  misc_feature 1..363: note = Synthetic
  source 1..363: mol_type = other DNA
gaggtgcagctggtggagtctgggggaggcttggtccagcctggggggtccctgagactctcctgtacagcctctggattcatttttagtaacttttggatgacttgggtccgccaggctccagggaaggggctggagtgggtggccaacataaagcaagatggaagtgagacatactgtgtggactctgtgaagggccgattcaccatctccagagaccacgccaagaactcactgtttctgcaaatgaacagcctgagagccgaggacacggctgtatattactgtgcaagaggagctggaacaatctactactacggtatggacgtctggggccaagggaccacggtcattgtctcctca

SEQ ID NO: 2 - protein, 121 aa, synthetic construct
  REGION 1..121: note = Synthetic
EVQLVESGGGLVQPGGSLRLSCTASGFIFSNFWMTWVRQAPGKGLEWVANIKQDGSETYCVDSVKGRFTISRDHAKNSLFLQMNSLRAEDTAVYYCARGAGTIYYYGMDVWGQGTTVIVSS

SEQ ID NO: 3 - DNA, 24 bp, synthetic construct
  misc_feature 1..24: note = Synthetic
  source 1..24: mol_type = other DNA
ggattcatttttagtaacttttgg

SEQ ID NO: 4 - protein, 8 aa, synthetic construct
  REGION 1..8: note = Synthetic
GFIFSNFW

SEQ ID NO: 5 - DNA, 24 bp, synthetic construct
  misc_feature 1..24: note = Synthetic
  source 1..24: mol_type = other DNA
ataaagcaagatggaagtgagaca

SEQ ID NO: 6 - protein, 8 aa, synthetic construct
  REGION 1..8: note = Synthetic
IKQDGSET

SEQ ID NO: 7 - DNA, 42 bp, synthetic construct
  misc_feature 1..42: note = Synthetic
  source 1..42: mol_type = other DNA
gcaagaggagctggaacaatctactactacggtatggacgtc

SEQ ID NO: 8 - protein, 14 aa, synthetic construct
  REGION 1..14: note = Synthetic
ARGAGTIYYYGMDV

SEQ ID NO: 9 - DNA, 321 bp, synthetic construct
  misc_feature 1..321: note = Synthetic
  source 1..321: mol_type = other DNA
gacatccagatgacccagtctccatcttccgtgtctgcatctgtaggagacagactcaccatcacttgtcgggcgagtcaggatattagcagctggttaacctggtatcagcagaaaccagggaaagcccctaacctcctgatctatgctgcatccggtttgcaaagtggagtcccatcaaggttcagcggcagtggatctgggacagatttcactctcaccatcagcaacctgcagcctgaagattttgcaacttactattgtcaacaggctaacagtttcccgctcaccttcggccaagggacacgactggagattaaa

SEQ ID NO: 10 - protein, 107 aa, synthetic construct
  REGION 1..107: note = Synthetic
DIQMTQSPSSVSASVGDRLTITCRASQDISSWLTWYQQKPGKAPNLLIYAASGLQSGVPSRFSGSGSGTDFTLTISNLQPEDFATYYCQQANSFPLTFGQGTRLEIK

SEQ ID NO: 11 - DNA, 18 bp, synthetic construct
  misc_feature 1..18: note = Synthetic
  source 1..18: mol_type = other DNA
caggatattagcagctgg

SEQ ID NO: 12 - protein, 6 aa, synthetic construct
  REGION 1..6: note = Synthetic
QDISSW

SEQ ID NO: 13-14 - skipped (2 entries)

SEQ ID NO: 15 - DNA, 27 bp, synthetic construct
  misc_feature 1..27: note = Synthetic
  source 1..27: mol_type = other DNA
caacaggctaacagtttcccgctcacc

SEQ ID NO: 16 - protein, 9 aa, synthetic construct
  REGION 1..9: note = Synthetic
QQANSFPLT

SEQ ID NO: 17 - DNA, 357 bp, synthetic construct
  misc_feature 1..357: note = Synthetic
  source 1..357: mol_type = other DNA
gaggtgcagctggtggagtctgggggaggcctggtcaagcctggggggtccctgagactctcctgtgcagcctctggattcaccttcagaaactataacataaactgggtccgccaggctccagggaaggggctggagtgggtctcactcatcagtggtagtagtagttacatatattacgcagactcagtgaagggccgattcaccgtctccagagacaacgccaagaactcactgtatctgcaaatgaacagcctgagagccgaggacacggctgtgtattactgtgcgaggcggacattaagctactacgttatggacgtctggggccaagggaccacggtcaccgtctcctca

SEQ ID NO: 18 - protein, 119 aa, synthetic construct
  REGION 1..119: note = Synthetic
EVQLVESGGGLVKPGGSLRLSCAASGFTFRNYNINWVRQAPGKGLEWVSLISGSSSYIYYADSVKGRFTVSRDNAKNSLYLQMNSLRAEDTAVYYCARRTLSYYVMDVWGQGTTVTVSS

SEQ ID NO: 19 - DNA, 24 bp, synthetic construct
  misc_feature 1..24: note = Synthetic
  source 1..24: mol_type = other DNA
ggattcaccttcagaaactataac

SEQ ID NO: 20 - protein, 8 aa, synthetic construct
  REGION 1..8: note = Synthetic
GFTFRNYN

SEQ ID NO: 21 - DNA, 24 bp, synthetic construct
  misc_feature 1..24: note = Synthetic
  source 1..24: mol_type = other DNA
atcagtggtagtagtagttacata

SEQ ID NO: 22 - protein, 8 aa, synthetic construct
  REGION 1..8: note = Synthetic
ISGSSSYI

SEQ ID NO: 23 - DNA, 36 bp, synthetic construct
  misc_feature 1..36: note = Synthetic
  source 1..36: mol_type = other DNA
gcgaggcggacattaagctactacgttatggacgtc

SEQ ID NO: 24 - protein, 12 aa, synthetic construct
  REGION 1..12: note = Synthetic
ARRTLSYYVMDV

SEQ ID NO: 25 - DNA, 321 bp, synthetic construct
  misc_feature 1..321: note = Synthetic
  source 1..321: mol_type = other DNA
gacatccaggtgacccagtctccatcccccctgtctgcatctgtaggagacagagtcaccatcacttgccgggcgagtcagggcattagcaattatttagcctggtatcagcagaaaccagggagagttcctcagctcctgatctatgctgcatccactttgcaatcaggggtcccatctcggttcagtggcagtggatctgggacagatttcactctcaccatcagcagcctgcagcctgaagatgttgcaacttattactgtcaaaagtataacagtgccccgtacacttttggccaggggaccaagctggagatcaaa

SEQ ID NO: 26 - protein, 107 aa, synthetic construct
  REGION 1..107: note = Synthetic
DIQVTQSPSPLSASVGDRVTITCRASQGISNYLAWYQQKPGRVPQLLIYAASTLQSGVPSRFSGSGSGTDFTLTISSLQPEDVATYYCQKYNSAPYTFGQGTKLEIK

SEQ ID NO: 27 - DNA, 18 bp, synthetic construct
  misc_feature 1..18: note = Synthetic
  source 1..18: mol_type = other DNA
cagggcattagcaattat

SEQ ID NO: 28 - protein, 6 aa, synthetic construct
  REGION 1..6: note = Synthetic
QGISNY

SEQ ID NO: 29-30 - skipped (2 entries)

SEQ ID NO: 31 - DNA, 27 bp, synthetic construct
  misc_feature 1..27: note = Synthetic
  source 1..27: mol_type = other DNA
caaaagtataacagtgccccgtacact

SEQ ID NO: 32 - protein, 9 aa, synthetic construct
  REGION 1..9: note = Synthetic
QKYNSAPYT

SEQ ID NO: 33 - DNA, 363 bp, synthetic construct
  misc_feature 1..363: note = Synthetic
  source 1..363: mol_type = other DNA
caggtacagctgcagcagtcaggtccaggactggtgaagtcctcgcagaccctctcactcacctgtgccatctccggggacagtgtctctagcaacagtgttgcttggaattggatcaggcagtccccatcgagaggccttgagtggctggggaggacatactacaggtccaaatggtataatgattatgcagtatctgtgaaaagtcgaataaacatcaacccagacacatccaagaaccacttctccctgcagttgaattctgtgactcccgaggacacggctgtttatttctgtgcaagagcctggaactggtactaccttgactactggggccagggcaccctggtcaccgtctcgtca

SEQ ID NO: 34 - protein, 121 aa, synthetic construct
  REGION 1..121: note = Synthetic
QVQLQQSGPGLVKSSQTLSLTCAISGDSVSSNSVAWNWIRQSPSRGLEWLGRTYYRSKWYNDYAVSVKSRININPDTSKNHFSLQLNSVTPEDTAVYFCARAWNWYYLDYWGQGTLVTVSS

SEQ ID NO: 35 - DNA, 30 bp, synthetic construct
  misc_feature 1..30: note = Synthetic
  source 1..30: mol_type = other DNA
ggggacagtgtctctagcaacagtgttgct

SEQ ID NO: 36 - protein, 10 aa, synthetic construct
  REGION 1..10: note = Synthetic
GDSVSSNSVA

SEQ ID NO: 37 - DNA, 27 bp, synthetic construct
  misc_feature 1..27: note = Synthetic
  source 1..27: mol_type = other DNA
acatactacaggtccaaatggtataat

SEQ ID NO: 38 - protein, 9 aa, synthetic construct
  REGION 1..9: note = Synthetic
TYYRSKWYN

SEQ ID NO: 39 - DNA, 33 bp, synthetic construct
  misc_feature 1..33: note = Synthetic
  source 1..33: mol_type = other DNA
gcaagagcctggaactggtactaccttgactac

SEQ ID NO: 40 - protein, 11 aa, synthetic construct
  REGION 1..11: note = Synthetic
ARAWNWYYLDY

SEQ ID NO: 41 - DNA, 339 bp, synthetic construct
  misc_feature 1..339: note = Synthetic
  source 1..339: mol_type = other DNA
gatattgtgatgacccagtctccagactccctggctatgtctctaggcgagagggccaccatcaactgcaagtccagccagagtgttttatacagctccaacaataagaattacttaggttggtaccagcagaaaccaggacagcctcctaaactgctcatttactgggcatctacccgggaatccggtgtccctgaccgaatcagtggcagcgggtctgggacagatttcactctcaccatcagcagcctgcaggctgaagatgtggcagtttattactgtcagcaatatcttagaaatacgctcactttcggcggagggaccaaggtggagatcaaa

SEQ ID NO: 42 - protein, 113 aa, synthetic construct
  REGION 1..113: note = Synthetic
DIVMTQSPDSLAMSLGERATINCKSSQSVLYSSNNKNYLGWYQQKPGQPPKLLIYWASTRESGVPDRISGSGSGTDFTLTISSLQAEDVAVYYCQQYLRNTLTFGGGTKVEIK

SEQ ID NO: 43 - DNA, 36 bp, synthetic construct
  misc_feature 1..36: note = Synthetic
  source 1..36: mol_type = other DNA
cagagtgttttatacagctccaacaataagaattac

SEQ ID NO: 44 - protein, 12 aa, synthetic construct
  REGION 1..12: note = Synthetic
QSVLYSSNNKNY

SEQ ID NO: 45-46 - skipped (2 entries)

SEQ ID NO: 47 - DNA, 27 bp, synthetic construct
  misc_feature 1..27: note = Synthetic
  source 1..27: mol_type = other DNA
cagcaatatcttagaaatacgctcact

SEQ ID NO: 48 - protein, 9 aa, synthetic construct
  REGION 1..9: note = Synthetic
QQYLRNTLT

SEQ ID NO: 49 - DNA, 381 bp, synthetic construct
  misc_feature 1..381: note = Synthetic
  source 1..381: mol_type = other DNA
gaggtgcagctggtggagtctgggggaggcctggtcaagcctggggggtccctgagactctcctgtgcagcctctggattcaccttcagtagctatagcatgaactgggtccgccaggctccagggaaggggctggagtgggtctcatccattagtagtagaagtagttacatatactacgcagactcagtgaagggccgattcaccatctcaagagacaacgccaagaactcactgtatctgcaaatgaacagcctgagagccgaggacacggctgtgtattattgtgcgagagatcatattgtagtagtaccaggtgcctcctactactactacggtatggacgtctggggccaagggaccacggtcaccgtctcctca

SEQ ID NO: 50 - protein, 127 aa, synthetic construct
  REGION 1..127: note = Synthetic
EVQLVESGGGLVKPGGSLRLSCAASGFTFSSYSMNWVRQAPGKGLEWVSSISSRSSYIYYADSVKGRFTISRDNAKNSLYLQMNSLRAEDTAVYYCARDHIVVVPGASYYYYGMDVWGQGTTVTVSS

SEQ ID NO: 51 - DNA, 24 bp, synthetic construct
  misc_feature 1..24: note = Synthetic
  source 1..24: mol_type = other DNA
ggattcaccttcagtagctatagc

SEQ ID NO: 52 - protein, 8 aa, synthetic construct
  REGION 1..8: note = Synthetic
GFTFSSYS

SEQ ID NO: 53 - DNA, 24 bp, synthetic construct
  misc_feature 1..24: note = Synthetic
  source 1..24: mol_type = other DNA
attagtagtagaagtagttacata

SEQ ID NO: 54 - protein, 8 aa, synthetic construct
  REGION 1..8: note = Synthetic
ISSRSSYI

SEQ ID NO: 55 - DNA, 60 bp, synthetic construct
  misc_feature 1..60: note = Synthetic
  source 1..60: mol_type = other DNA
gcgagagatcatattgtagtagtaccaggtgcctcctactactactacggtatggacgtc

SEQ ID NO: 56 - protein, 20 aa, synthetic construct
  REGION 1..20: note = Synthetic
ARDHIVVVPGASYYYYGMDV

SEQ ID NO: 57 - DNA, 321 bp, synthetic construct
  misc_feature 1..321: note = Synthetic
  source 1..321: mol_type = other DNA
gacatccagatgacccagtctccatcctccctgtctgcatctgtaggagacagagtcaccatcacttgccgggcaagtcagggcattagaaatgatttaggctggtatcagcagaaaccagggaaagcccctaagcgcctgatctctgctgcatccagtttgcaaagtggggtcccatcaaggttcagcggcagtggatctgggacagaattcactctcacaatcagcagcctgcagcctgaagattttgcaacttattactgtctacagcataatagttacccgctcactttcggcggagggaccaaggtggagatcaaa

SEQ ID NO: 58 - protein, 107 aa, synthetic construct
  REGION 1..107: note = Synthetic
DIQMTQSPSSLSASVGDRVTITCRASQGIRNDLGWYQQKPGKAPKRLISAASSLQSGVPSRFSGSGSGTEFTLTISSLQPEDFATYYCLQHNSYPLTFGGGTKVEIK

SEQ ID NO: 59 - DNA, 18 bp, synthetic construct
  misc_feature 1..18: note = Synthetic
  source 1..18: mol_type = other DNA
cagggcattagaaatgat

SEQ ID NO: 60 - protein, 6 aa, synthetic construct
  REGION 1..6: note = Synthetic
QGIRND

SEQ ID NO: 61-62 - skipped (2 entries)

SEQ ID NO: 63 - DNA, 27 bp, synthetic construct
  misc_feature 1..27: note = Synthetic
  source 1..27: mol_type = other DNA
ctacagcataatagttacccgctcact

SEQ ID NO: 64 - protein, 9 aa, synthetic construct
  REGION 1..9: note = Synthetic
LQHNSYPLT

SEQ ID NO: 65 - DNA, 369 bp, synthetic construct
  misc_feature 1..369: note = Synthetic
  source 1..369: mol_type = other DNA
caggtgcagctggtgcagtctggggctgaggtgaagaagcctggggcctcagtggaggtctcctgcaaggcttctggatacaccttcaccgactactatatacactggatacgacaggcccctggacaagggcttgagtggatgggatggatcaaccctgacagtggtcgcacaaactatgcacagaagtttcaggtcagggtcaccatgaccagggacacgtccatcaccacagcctacatggaactgaacagactgaaatctgacgacacggccgtgtattactgtgcgagaggacccctacgtggatatagcggctacgatttttttgactactggggccagggaaccctggtcaccgtctcctca

SEQ ID NO: 66 - protein, 123 aa, synthetic construct
  REGION 1..123: note = Synthetic
QVQLVQSGAEVKKPGASVEVSCKASGYTFTDYYIHWIRQAPGQGLEWMGWINPDSGRTNYAQKFQVRVTMTRDTSITTAYMELNRLKSDDTAVYYCARGPLRGYSGYDFFDYWGQGTLVTVSS

SEQ ID NO: 67 - DNA, 24 bp, synthetic construct
  misc_feature 1..24: note = Synthetic
  source 1..24: mol_type = other DNA
ggatacaccttcaccgactactat

SEQ ID NO: 68 - protein, 8 aa, synthetic construct
  REGION 1..8: note = Synthetic
GYTFTDYY

SEQ ID NO: 69 - DNA, 24 bp, synthetic construct
  misc_feature 1..24: note = Synthetic
  source 1..24: mol_type = other DNA
atcaaccctgacagtggtcgcaca

SEQ ID NO: 70 - protein, 8 aa, synthetic construct
  REGION 1..8: note = Synthetic
INPDSGRT

SEQ ID NO: 71 - DNA, 48 bp, synthetic construct
  misc_feature 1..48: note = Synthetic
  source 1..48: mol_type = other DNA
gcgagaggacccctacgtggatatagcggctacgatttttttgactac

SEQ ID NO: 72 - protein, 16 aa, synthetic construct
  REGION 1..16: note = Synthetic
ARGPLRGYSGYDFFDY

SEQ ID NO: 73 - DNA, 339 bp, synthetic construct
  misc_feature 1..339: note = Synthetic
  source 1..339: mol_type = other DNA
gacatcgtgatgacccagtctccagactccctggctatatctctgggcgagagggccaccatcaactgcaagtccagccagagtgttttatacagctccaacaataagcagtacttagcttggtacaagcagagaccaggacagcctcctaagctgctcatttcctggacatctacccgggaatccggggtccctgaccgattcagtggcagcgggtctgggacagatttcactctcaccatcagcagcctgcaggctgaagatgtggcagtttatttctgtcaacaatattatagtactccgtacacttttggccaggggaccaagctggagatcaga

SEQ ID NO: 74 - protein, 113 aa, synthetic construct
  REGION 1..113: note = Synthetic
DIVMTQSPDSLAISLGERATINCKSSQSVLYSSNNKQYLAWYKQRPGQPPKLLISWTSTRESGVPDRFSGSGSGTDFTLTISSLQAEDVAVYFCQQYYSTPYTFGQGTKLEIR

SEQ ID NO: 75 - DNA, 36 bp, synthetic construct
  misc_feature 1..36: note = Synthetic
  source 1..36: mol_type = other DNA
cagagtgttttatacagctccaacaataagcagtac

SEQ ID NO: 76 - protein, 12 aa, synthetic construct
  REGION 1..12: note = Synthetic
QSVLYSSNNKQY

SEQ ID NO: 77-78 - skipped (2 entries)

SEQ ID NO: 79 - DNA, 27 bp, synthetic construct
  misc_feature 1..27: note = Synthetic
  source 1..27: mol_type = other DNA
caacaatattatagtactccgtacact

SEQ ID NO: 80 - protein, 9 aa, synthetic construct
  REGION 1..9: note = Synthetic
QQYYSTPYT

SEQ ID NO: 81 - DNA, 369 bp, synthetic construct
  misc_feature 1..369: note = Synthetic
  source 1..369: mol_type = other DNA
caggtggtactggtggagtctgggggaggcgtggtccagcctgggaggtccctgagactctcctgtgcagcgtctggattcaccttcagtagctatggcatgcactgggtccgccaggctccaggcaaggggctggagtgggtggcagttatatggtatgatggaagtaataaatactatgtagactccgtgaagggccgattcaccatctccagagacaattccaataacacaatctatctgcaaatgaacagcctgagagccgaggacacggctgtatattactgtgcgagatcccttataccagtggctggtacggaccccatttttggatactggggccagggaaccctggtcaccgtctcctca

SEQ ID NO: 82 - protein, 123 aa, synthetic construct
  REGION 1..123: note = Synthetic
QVVLVESGGGVVQPGRSLRLSCAASGFTFSSYGMHWVRQAPGKGLEWVAVIWYDGSNKYYVDSVKGRFTISRDNSNNTIYLQMNSLRAEDTAVYYCARSLIPVAGTDPIFGYWGQGTLVTVSS

SEQ ID NO: 83 - DNA, 24 bp, synthetic construct
  misc_feature 1..24: note = Synthetic
  source 1..24: mol_type = other DNA
ggattcaccttcagtagctatggc

SEQ ID NO: 84 - protein, 8 aa, synthetic construct
  REGION 1..8: note = Synthetic
GFTFSSYG

SEQ ID NO: 85 - DNA, 24 bp, synthetic construct
  misc_feature 1..24: note = Synthetic
  source 1..24: mol_type = other DNA
atatggtatgatggaagtaataaa

SEQ ID NO: 86 - protein, 8 aa, synthetic construct
  REGION 1..8: note = Synthetic
IWYDGSNK

SEQ ID NO: 87 - DNA, 48 bp, synthetic construct
  misc_feature 1..48: note = Synthetic
  source 1..48: mol_type = other DNA
gcgagatcccttataccagtggctggtacggaccccatttttggatac

SEQ ID NO: 88 - protein, 16 aa, synthetic construct
  REGION 1..16: note = Synthetic
ARSLIPVAGTDPIFGY

SEQ ID NO: 89 - DNA, 321 bp, synthetic construct
  misc_feature 1..321: note = Synthetic
  source 1..321: mol_type = other DNA
gacatccagatgacccagtctccttccaccctgtctgcatctgtaggagacagagtcaccatcacttgccgggccagtcagagtgttagtagctggttggcctggtatcagcagaaaccagggaaagcccctaaactcctgatctttaaggcgtctggtttagaaagtggggtcccatttaggttcagcggcagtggatctgggacagaattcactctcaccatcagcagcctgcagcctgatgattttgcaacttattactgccaacagtataatacttattctccgacgttcggccaagggaccaaggtggagatcaaa

SEQ ID NO: 90 - protein, 107 aa, synthetic construct
  REGION 1..107: note = Synthetic
DIQMTQSPSTLSASVGDRVTITCRASQSVSSWLAWYQQKPGKAPKLLIFKASGLESGVPFRFSGSGSGTEFTLTISSLQPDDFATYYCQQYNTYSPTFGQGTKVEIK

SEQ ID NO: 91 - DNA, 18 bp, synthetic construct
  misc_feature 1..18: note = Synthetic
  source 1..18: mol_type = other DNA
cagagtgttagtagctgg

SEQ ID NO: 92 - protein, 6 aa, synthetic construct
  REGION 1..6: note = Synthetic
QSVSSW

SEQ ID NO: 93-94 - skipped (2 entries)

SEQ ID NO: 95 - DNA, 27 bp, synthetic construct
  misc_feature 1..27: note = Synthetic
  source 1..27: mol_type = other DNA
caacagtataatacttattctccgacg

SEQ ID NO: 96 - protein, 9 aa, synthetic construct
  REGION 1..9: note = Synthetic
QQYNTYSPT

SEQ ID NO: 97 - DNA, 360 bp, synthetic construct
  misc_feature 1..360: note = Synthetic
  source 1..360: mol_type = other DNA
caggtgcagctgcaggagtcgggcccaggactggtgaagccttcggagaccctgtccctcacctgcactgtctctggtggctccatcagtaattactactggagctggatccggcagcccccagggaagggactggagtggattggatatatctattatagtgggagaaccaactacaacccctccctcaagagtcgagtcaccatatcagtggacacgtccaagaaccagttctccctgaagctgaggtctgtgaccgccgcagacacggccgtgtattactgtgcgagacatcgtataactagaactgcggactcctttgactactggggccagggaaccctggtcaccgtctcctca

SEQ ID NO: 98 - protein, 120 aa, synthetic construct
  REGION 1..120: note = Synthetic
QVQLQESGPGLVKPSETLSLTCTVSGGSISNYYWSWIRQPPGKGLEWIGYIYYSGRTNYNPSLKSRVTISVDTSKNQFSLKLRSVTAADTAVYYCARHRITRTADSFDYWGQGTLVTVSS

SEQ ID NO: 99 - DNA, 24 bp, synthetic construct
  misc_feature 1..24: note = Synthetic
  source 1..24: mol_type = other DNA
ggtggctccatcagtaattactac

SEQ ID NO: 100 - protein, 8 aa, synthetic construct
  REGION 1..8: note = Synthetic
GGSISNYY

SEQ ID NO: 101 - DNA, 21 bp, synthetic construct
  misc_feature 1..21: note = Synthetic
  source 1..21: mol_type = other DNA
atctattatagtgggagaacc

SEQ ID NO: 102 - protein, 7 aa, synthetic construct
  REGION 1..7: note = Synthetic
IYYSGRT

SEQ ID NO: 103 - DNA, 42 bp, synthetic construct
  misc_feature 1..42: note = Synthetic
  source 1..42: mol_type = other DNA
gcgagacatcgtataactagaactgcggactcctttgactac

SEQ ID NO: 104 - protein, 14 aa, synthetic construct
  REGION 1..14: note = Synthetic
ARHRITRTADSFDY

SEQ ID NO: 105 - DNA, 321 bp, synthetic construct
  misc_feature 1..321: note = Synthetic
  source 1..321: mol_type = other DNA
gacatccagatgacccagtctccatcctccctgtctgcatctgtaggagacagagtcaccatcacttgccaggcgagtcaggacattaccaactatttaaattggtatcagcagaaaccagggaaagcccctaagctcctgatctacgatgcatccaatttggaaacaggggtcccatcaaggttcagtggaagtggatctgggacagattttactttcaccatcagcagcctgcagcctgaagatgttgcaacattttactgtcaccagtatggtgatctcccgtacacttttggccaggggaccaagctggagatcaaa

SEQ ID NO: 106 - protein, 107 aa, synthetic construct
  REGION 1..107: note = Synthetic
DIQMTQSPSSLSASVGDRVTITCQASQDITNYLNWYQQKPGKAPKLLIYDASNLETGVPSRFSGSGSGTDFTFTISSLQPEDVATFYCHQYGDLPYTFGQGTKLEIK

SEQ ID NO: 107 - DNA, 18 bp, synthetic construct
  misc_feature 1..18: note = Synthetic
  source 1..18: mol_type = other DNA
caggacattaccaactat

SEQ ID NO: 108 - protein, 6 aa, synthetic construct
  REGION 1..6: note = Synthetic
QDITNY

SEQ ID NO: 109-110 - skipped (2 entries)

SEQ ID NO: 111 - DNA, 27 bp, synthetic construct
  misc_feature 1..27: note = Synthetic
  source 1..27: mol_type = other DNA
caccagtatggtgatctcccgtacact

SEQ ID NO: 112 - protein, 9 aa, synthetic construct
  REGION 1..9: note = Synthetic
HQYGDLPYT

SEQ ID NO: 113 - DNA, 369 bp, synthetic construct
  misc_feature 1..369: note = Synthetic
  source 1..369: mol_type = other DNA
caggtggtattggtggagtctgggggaggcgtggtccagcctgggaggtccctgagactctcctgtgcagcgtctggattcaccttcagtagctatggcatgcactgggtccgccaggctccaggcaaggggctggagtgggtggcagttatttggtatgatggaagtattaaatactatgcagactccgtgaagggccgattcaccatctccagagacaattccaataacacaatctatctgcaaatgaacagcctgagagccgaggacacggctgtatattactgtgcgagagcccttataccagtggctggtacggaccccatttttgggtactggggccagggaaccctggtcaccgtctcctca

SEQ ID NO: 114 - protein, 123 aa, synthetic construct
  REGION 1..123: note = Synthetic
QVVLVESGGGVVQPGRSLRLSCAASGFTFSSYGMHWVRQAPGKGLEWVAVIWYDGSIKYYADSVKGRFTISRDNSNNTIYLQMNSLRAEDTAVYYCARALIPVAGTDPIFGYWGQGTLVTVSS

SEQ ID NO: 115 - DNA, 24 bp, synthetic construct
  misc_feature 1..24: note = Synthetic
  source 1..24: mol_type = other DNA
ggattcaccttcagtagctatggc

SEQ ID NO: 116 - protein, 8 aa, synthetic construct
  REGION 1..8: note = Synthetic
GFTFSSYG

SEQ ID NO: 117 - DNA, 24 bp, synthetic construct
  misc_feature 1..24: note = Synthetic
  source 1..24: mol_type = other DNA
atttggtatgatggaagtattaaa

SEQ ID NO: 118 - protein, 8 aa, synthetic construct
  REGION 1..8: note = Synthetic
IWYDGSIK

SEQ ID NO: 119 - DNA, 48 bp, synthetic construct
  misc_feature 1..48: note = Synthetic
  source 1..48: mol_type = other DNA
gcgagagcccttataccagtggctggtacggaccccatttttgggtac

SEQ ID NO: 120 - protein, 16 aa, synthetic construct
  REGION 1..16: note = Synthetic
ARALIPVAGTDPIFGY

SEQ ID NO: 121 - DNA, 321 bp, synthetic construct
  misc_feature 1..321: note = Synthetic
  source 1..321: mol_type = other DNA
gacatccagatgacccagtctccttccaccctgtctgcatctgtaggagacagagtcaccatcacttgccgggccagtcagagtgttagtagctggttggcctggtatcagcagaaaccagggaaagcccctaaactcctgatctttaagacgtctggtttagaaagtggggtcccatttaggttcagcggcagtggatctgggacagaattcactctcaccatcagcagcctgcagcctgatgattttgcaacttattactgccaacagtataatacttattctccgacgttcggccaagggaccaaggtggagatcaaa

SEQ ID NO: 122 - protein, 107 aa, synthetic construct
  REGION 1..107: note = Synthetic
DIQMTQSPSTLSASVGDRVTITCRASQSVSSWLAWYQQKPGKAPKLLIFKTSGLESGVPFRFSGSGSGTEFTLTISSLQPDDFATYYCQQYNTYSPTFGQGTKVEIK

SEQ ID NO: 123 - DNA, 18 bp, synthetic construct
  misc_feature 1..18: note = Synthetic
  source 1..18: mol_type = other DNA
cagagtgttagtagctgg

SEQ ID NO: 124 - protein, 6 aa, synthetic construct
  REGION 1..6: note = Synthetic
QSVSSW

SEQ ID NO: 125-126 - skipped (2 entries)

SEQ ID NO: 127 - DNA, 27 bp, synthetic construct
  misc_feature 1..27: note = Synthetic
  source 1..27: mol_type = other DNA
caacagtataatacttattctccgacg

SEQ ID NO: 128 - protein, 9 aa, synthetic construct
  REGION 1..9: note = Synthetic
QQYNTYSPT

SEQ ID NO: 129 - DNA, 360 bp, synthetic construct
  misc_feature 1..360: note = Synthetic
  source 1..360: mol_type = other DNA
caggtgcagctgcaggagtcgggcccaggactggtgaagccttcggagaccctgtccctcacctgcactgtctctggtggctccatcagtagttactactggagctggatccggcagcccccagggaagggactggagtggattggatatatctattacagtgggagaaccaactacaacccctccctcaagagtcgagtcaccatatcagtggacacgtccaagaaccagttctccctgaaactgagctctgtgaccgccgcagacacggccatttattactgtgcgagacatcgtgtaactagaactgcggactcctttgactactggggccagggaaccctggtcaccgtctcctca

SEQ ID NO: 130 - protein, 120 aa, synthetic construct
  REGION 1..120: note = Synthetic
QVQLQESGPGLVKPSETLSLTCTVSGGSISSYYWSWIRQPPGKGLEWIGYIYYSGRTNYNPSLKSRVTISVDTSKNQFSLKLSSVTAADTAIYYCARHRVTRTADSFDYWGQGTLVTVSS

SEQ ID NO: 131 - DNA, 24 bp, synthetic construct
  misc_feature 1..24: note = Synthetic
  source 1..24: mol_type = other DNA
ggtggctccatcagtagttactac

SEQ ID NO: 132 - protein, 8 aa, synthetic construct
  REGION 1..8: note = Synthetic
GGSISSYY

SEQ ID NO: 133 - DNA, 21 bp, synthetic construct
  misc_feature 1..21: note = Synthetic
  source 1..21: mol_type = other DNA
atctattacagtgggagaacc

SEQ ID NO: 134 - protein, 7 aa, synthetic construct
  REGION 1..7: note = Synthetic
IYYSGRT

SEQ ID NO: 135 - DNA, 42 bp, synthetic construct
  misc_feature 1..42: note = Synthetic
  source 1..42: mol_type = other DNA
gcgagacatcgtgtaactagaactgcggactcctttgactac

SEQ ID NO: 136 - protein, 14 aa, synthetic construct
  REGION 1..14: note = Synthetic
ARHRVTRTADSFDY

SEQ ID NO: 137 - DNA, 321 bp, synthetic construct
  misc_feature 1..321: note = Synthetic
  source 1..321: mol_type = other DNA
gacatccagatgacccagtctccatcctccctgtctgcatctgtaggagacagagtcaccatcacttgccaggcgagtcaggacattaacaactatttaaattggtatcagcagaaaacagggaaagcccctaagttcctgatctacgatgcatccaatttggaaacaggggtctcatcaaggttcagtggaagtggatctgggacagattttactttcaccatcagcagcctgcagcctgaagatgttggaacatattactgtcaccagtatggtgatctcccgtacacttttggccaggggaccaagctggagatcaaa

SEQ ID NO: 138 - protein, 107 aa, synthetic construct
  REGION 1..107: note = Synthetic
DIQMTQSPSSLSASVGDRVTITCQASQDINNYLNWYQQKTGKAPKFLIYDASNLETGVSSRFSGSGSGTDFTFTISSLQPEDVGTYYCHQYGDLPYTFGQGTKLEIK

SEQ ID NO: 139 - DNA, 18 bp, synthetic construct
  misc_feature 1..18: note = Synthetic
  source 1..18: mol_type = other DNA
caggacattaacaactat

SEQ ID NO: 140 - protein, 6 aa, synthetic construct
  REGION 1..6: note = Synthetic
QDINNY

SEQ ID NO: 141-142 - skipped (2 entries)

SEQ ID NO: 143 - DNA, 27 bp, synthetic construct
  misc_feature 1..27: note = Synthetic
  source 1..27: mol_type = other DNA
caccagtatggtgatctcccgtacact

SEQ ID NO: 144 - protein, 9 aa, synthetic construct
  REGION 1..9: note = Synthetic
HQYGDLPYT

SEQ ID NO: 145 - DNA, 360 bp, synthetic construct
  misc_feature 1..360: note = Synthetic
  source 1..360: mol_type = other DNA
gaggtgcagctggtggagtctgggggaggcctggtcaggccggggggatccctgagactctcctgtgcagcctctggattcaccttcactagctatgccatgaattgggtccgccaggctccagggaagggactggagtgggtctcatccatttctagttatagttcttacatatatatcgcagactcagtgaagggccgattcaccctctccagagacaatgccaagaactcactgtatctacaaatgcacagtctgagacccgaggacacggctgtttatttctgtgcgagagagggatatagtgcctactcctactttgacttctggggccggggaaccctggtcaccgtctcctca

SEQ ID NO: 146 - protein, 120 aa, synthetic construct
  REGION 1..120: note = Synthetic
EVQLVESGGGLVRPGGSLRLSCAASGFTFTSYAMNWVRQAPGKGLEWVSSISSYSSYIYIADSVKGRFTLSRDNAKNSLYLQMHSLRPEDTAVYFCAREGYSAYSYFDFWGRGTLVTVSS

SEQ ID NO: 147 - DNA, 24 bp, synthetic construct
  misc_feature 1..24: note = Synthetic
  source 1..24: mol_type = other DNA
ggattcaccttcactagctatgcc

SEQ ID NO: 148 - protein, 8 aa, synthetic construct
  REGION 1..8: note = Synthetic
GFTFTSYA

SEQ ID NO: 149 - DNA, 24 bp, synthetic construct
  misc_feature 1..24: note = Synthetic
  source 1..24: mol_type = other DNA
atttctagttatagttcttacata

SEQ ID NO: 150 - protein, 8 aa, synthetic construct
  REGION 1..8: note = Synthetic
ISSYSSYI

SEQ ID NO: 151 - DNA, 39 bp, synthetic construct
  misc_feature 1..39: note = Synthetic
  source 1..39: mol_type = other DNA
gcgagagagggatatagtgcctactcctactttgacttc

SEQ ID NO: 152 - protein, 13 aa, synthetic construct
  REGION 1..13: note = Synthetic
AREGYSAYSYFDF

SEQ ID NO: 153 - DNA, 321 bp, synthetic construct
  misc_feature 1..321: note = Synthetic
  source 1..321: mol_type = other DNA
gacatccagatgacccagtctccttccaccctgtctgcatctgttggagacagagtcaccatcacttgccgggccagtcagagtgttattagttggttggcctggtatcaacagaaaccagggaaagcccctaaactcctgatccatagggcgtctagtttagaaagtggggtcccatcaaggttcagcggcagtggatctgggacagaattcactctcaccatcagcggcctgcagcctgatgattttgcaacttattactgtcaacagtataatacttattttccgacgttcggccaagggaccaaggtggaagtcaaa

SEQ ID NO: 154 - protein, 107 aa, synthetic construct
  REGION 1..107: note = Synthetic
DIQMTQSPSTLSASVGDRVTITCRASQSVISWLAWYQQKPGKAPKLLIHRASSLESGVPSRFSGSGSGTEFTLTISGLQPDDFATYYCQQYNTYFPTFGQGTKVEVK

SEQ ID NO: 155 - DNA, 18 bp, synthetic construct
  misc_feature 1..18: note = Synthetic
  source 1..18: mol_type = other DNA
cagagtgttattagttgg

SEQ ID NO: 156 - protein, 6 aa, synthetic construct
  REGION 1..6: note = Synthetic
QSVISW

SEQ ID NO: 157-158 - skipped (2 entries)

SEQ ID NO: 159 - DNA, 27 bp, synthetic construct
  misc_feature 1..27: note = Synthetic
  source 1..27: mol_type = other DNA
caacagtataatacttattttccgacg

SEQ ID NO: 160 - protein, 9 aa, synthetic construct
  REGION 1..9: note = Synthetic
QQYNTYFPT

SEQ ID NO: 161 - DNA, 354 bp, synthetic construct
  misc_feature 1..354: note = Synthetic
  source 1..354: mol_type = other DNA
gaggtggaactgttggaatctgggggaggcttggtacagcctggggggtccctgagactctcctgtgcagcctctggattcacctttagtagttatgccatgagttgggtccgccaggctccagggaaggggctggagtgggtctcatctattagtggtagggttggtagcacacatttcgcagactccgtgaagggccggttcaccttctccagagacaattccaagaacacgctgtatctgcagctgagcagcctgagagccgaggacacggccgtatattactgtgcgagaagtagaggagcagcctactttgactactggggccagggaaccctggtcaccgtctcctca

SEQ ID NO: 162 - protein, 118 aa, synthetic construct
  REGION 1..118: note = Synthetic
EVELLESGGGLVQPGGSLRLSCAASGFTFSSYAMSWVRQAPGKGLEWVSSISGRVGSTHFADSVKGRFTFSRDNSKNTLYLQLSSLRAEDTAVYYCARSRGAAYFDYWGQGTLVTVSS

SEQ ID NO: 163 - DNA, 24 bp, synthetic construct
  misc_feature 1..24: note = Synthetic
  source 1..24: mol_type = other DNA
ggattcacctttagtagttatgcc

SEQ ID NO: 164 - protein, 8 aa, synthetic construct
  REGION 1..8: note = Synthetic
GFTFSSYA

SEQ ID NO: 165 - DNA, 24 bp, synthetic construct
  misc_feature 1..24: note = Synthetic
  source 1..24: mol_type = other DNA
attagtggtagggttggtagcaca

SEQ ID NO: 166 - protein, 8 aa, synthetic construct
  REGION 1..8: note = Synthetic
ISGRVGST

SEQ ID NO: 167 - DNA, 33 bp, synthetic construct
  misc_feature 1..33: note = Synthetic
  source 1..33: mol_type = other DNA
gcgagaagtagaggagcagcctactttgactac

SEQ ID NO: 168 - protein, 11 aa, synthetic construct
  REGION 1..11: note = Synthetic
ARSRGAAYFDY

SEQ ID NO: 169 - DNA, 321 bp, synthetic construct
  misc_feature 1..321: note = Synthetic
  source 1..321: mol_type = other DNA
gacatccagatgacccagtctccatcctccctgtctgcatctgtaggagacagagtcaccatcacttgccaggcgaatcaggacattagcaactttttaaattggtatcagcagagaccagggaaagcccctaacctcctgatctatgctgcatccaatttggaaacaggggtcccatcaaggttcagtggaagtggatctgggacagattttactttcaccatcagcagcctgcagcctgaagatattgcaacatattactgtcaacattatgataattttccattcactttcggccctgggaccaaggtggatatcaaa

SEQ ID NO: 170 - protein, 107 aa, synthetic construct
  REGION 1..107: note = Synthetic
DIQMTQSPSSLSASVGDRVTITCQANQDISNFLNWYQQRPGKAPNLLIYAASNLETGVPSRFSGSGSGTDFTFTISSLQPEDIATYYCQHYDNFPFTFGPGTKVDIK

SEQ ID NO: 171 - DNA, 18 bp, synthetic construct
  misc_feature 1..18: note = Synthetic
  source 1..18: mol_type = other DNA
caggacattagcaacttt

SEQ ID NO: 172 - protein, 6 aa, synthetic construct
  REGION 1..6: note = Synthetic
QDISNF

SEQ ID NO: 173-174 - skipped (2 entries)

SEQ ID NO: 175 - DNA, 27 bp, synthetic construct
  misc_feature 1..27: note = Synthetic
  source 1..27: mol_type = other DNA
caacattatgataattttccattcact

SEQ ID NO: 176 - protein, 9 aa, synthetic construct
  REGION 1..9: note = Synthetic
QHYDNFPFT

SEQ ID NO: 177 - DNA, 363 bp, synthetic construct
  misc_feature 1..363: note = Synthetic
  source 1..363: mol_type = other DNA
cagctgcagctgcaggagtcgggcccaggactggtgaacccttcggagaccctgtccctcacctgctctgtctctggtggctccatcagcagtgttaattactactggggctggatccgccagtccccagggaagggactggagtggattgggagtatctattatactgggagtaccgactacaacccgtccctcaagaatcgagtcaccatatccgtagacacgtccaagaaccagttctccctgaagcagacttctgtgaccgccgcagacacggctgtctattactgtgcgagacatgtggcactggctgggggggcttttgatatctggggccaggggacaatggtcaccgtctcttca

SEQ ID NO: 178 - protein, 121 aa, synthetic construct
  REGION 1..121: note = Synthetic
QLQLQESGPGLVNPSETLSLTCSVSGGSISSVNYYWGWIRQSPGKGLEWIGSIYYTGSTDYNPSLKNRVTISVDTSKNQFSLKQTSVTAADTAVYYCARHVALAGGAFDIWGQGTMVTVSS

SEQ ID NO: 179 - DNA, 30 bp, synthetic construct
  misc_feature 1..30: note = Synthetic
  source 1..30: mol_type = other DNA
ggtggctccatcagcagtgttaattactac

SEQ ID NO: 180 - protein, 10 aa, synthetic construct
  REGION 1..10: note = Synthetic
GGSISSVNYY

SEQ ID NO: 181 - DNA, 21 bp, synthetic construct
  misc_feature 1..21: note = Synthetic
  source 1..21: mol_type = other DNA
atctattatactgggagtacc

SEQ ID NO: 182 - protein, 7 aa, synthetic construct
  REGION 1..7: note = Synthetic
IYYTGST

SEQ ID NO: 183 - DNA, 39 bp, synthetic construct
  misc_feature 1..39: note = Synthetic
  source 1..39: mol_type = other DNA
gcgagacatgtggcactggctgggggggcttttgatatc

SEQ ID NO: 184 - protein, 13 aa, synthetic construct
  REGION 1..13: note = Synthetic
ARHVALAGGAFDI

SEQ ID NO: 185 - DNA, 315 bp, synthetic construct
  misc_feature 1..315: note = Synthetic
  source 1..315: mol_type = other DNA
gaaattgtgttgacgcagtctccaggcaccctgtctttgtctccaggggaaagagccaccctctcctgcagggccagtcagagtgttagtagcagcttcttaggctggtaccaacagaaacctggccaggctcccaggctcctcatctatggttcttccaccagggccactggcatcccagacaggttcagtggcagtgggtctgggacagacttcaatatcaccatcagcagactggagcctgaagattttgcagtgtattactgtcagcagtttggtaggtccttcggccctgggaccaagctggagatcaaa

SEQ ID NO: 186 - protein, 105 aa, synthetic construct
  REGION 1..105: note = Synthetic
EIVLTQSPGTLSLSPGERATLSCRASQSVSSSFLGWYQQKPGQAPRLLIYGSSTRATGIPDRFSGSGSGTDFNITISRLEPEDFAVYYCQQFGRSFGPGTKLEIK

SEQ ID NO: 187 - DNA, 21 bp, synthetic construct
  misc_feature 1..21: note = Synthetic
  source 1..21: mol_type = other DNA
cagagtgttagtagcagcttc

SEQ ID NO: 188 - protein, 7 aa, synthetic construct
  REGION 1..7: note = Synthetic
QSVSSSF

SEQ ID NO: 189-190 - skipped (2 entries)

SEQ ID NO: 191 - DNA, 18 bp, synthetic construct
  misc_feature 1..18: note = Synthetic
  source 1..18: mol_type = other DNA
cagcagtttggtaggtcc

SEQ ID NO: 192 - protein, 6 aa, synthetic construct
  REGION 1..6: note = Synthetic
QQFGRS

SEQ ID NO: 193 - DNA, 360 bp, synthetic construct
  misc_feature 1..360: note = Synthetic
  source 1..360: mol_type = other DNA
caggtgcagctggtggagtctgggggaggcttggtcaagcctggagggtccctgagactctcctgcgcagcctctggattcaccttcagtgactattacatgaactggatccgccaggctccagggaaggggctggagtggatttcatatattagtagtggtggtagtaccacatactacgcagactctgtgaagggccgattcaccatctccagggacaacgccaagaactcactgtatctgcaaatgaacagcctgagagccgaggacacggccgtgtattactgtgcgagagatgggaagtacaacacctcgccgggggactactggggccagggaaccctggtcaccgtctcctca

SEQ ID NO: 194 - protein, 120 aa, synthetic construct
  REGION 1..120: note = Synthetic
QVQLVESGGGLVKPGGSLRLSCAASGFTFSDYYMNWIRQAPGKGLEWISYISSGGSTTYYADSVKGRFTISRDNAKNSLYLQMNSLRAEDTAVYYCARDGKYNTSPGDYWGQGTLVTVSS

SEQ ID NO: 195 - DNA, 24 bp, synthetic construct
  misc_feature 1..24: note = Synthetic
  source 1..24: mol_type = other DNA
ggattcaccttcagtgactattac

SEQ ID NO: 196 - protein, 8 aa, synthetic construct
  REGION 1..8: note = Synthetic
GFTFSDYY

SEQ ID NO: 197 - DNA, 24 bp, synthetic construct
  misc_feature 1..24: note = Synthetic
  source 1..24: mol_type = other DNA
attagtagtggtggtagtaccaca

SEQ ID NO: 198 - protein, 8 aa, synthetic construct
  REGION 1..8: note = Synthetic
ISSGGSTT

SEQ ID NO: 199 - DNA, 39 bp, synthetic construct
  misc_feature 1..39: note = Synthetic
  source 1..39: mol_type = other DNA
gcgagagatgggaagtacaacacctcgccgggggactac

SEQ ID NO: 200 - protein, 13 aa, synthetic construct
  REGION 1..13: note = Synthetic
ARDGKYNTSPGDY

SEQ ID NO: 201 - DNA, 318 bp, synthetic construct
  misc_feature 1..318: note = Synthetic
  source 1..318: mol_type = other DNA
gaaattgtgttgacgcagtctccagactttcagtctgtgactccaaaggagaaagtcaccatcacctgccgggccagtcagtccattggtagtagcttacactggtaccagcagaaaccagatcagtctccaaagctcctcatcaagtatgcttcccagtccttctcaggggtcccctcgaggttcagtggcagtggatctgggacagatttcaccctcaccatcaatagcctggaagctgaagatgctgctacgtattactgtcttcagagtagtagtttacggacgttcggccaagggaccaaagtggatatcaaa

SEQ ID NO: 202 - protein, 106 aa, synthetic construct
  REGION 1..106: note = Synthetic
EIVLTQSPDFQSVTPKEKVTITCRASQSIGSSLHWYQQKPDQSPKLLIKYASQSFSGVPSRFSGSGSGTDFTLTINSLEAEDAATYYCLQSSSLRTFGQGTKVDIK

SEQ ID NO: 203 - DNA, 18 bp, synthetic construct
  misc_feature 1..18: note = Synthetic
  source 1..18: mol_type = other DNA
cagtccattggtagtagc

SEQ ID NO: 204 - protein, 6 aa, synthetic construct
  REGION 1..6: note = Synthetic
QSIGSS

SEQ ID NO: 205-206 - skipped (2 entries)

SEQ ID NO: 207 - DNA, 24 bp, synthetic construct
  misc_feature 1..24: note = Synthetic
  source 1..24: mol_type = other DNA
cttcagagtagtagtttacggacg

SEQ ID NO: 208 - protein, 8 aa, synthetic construct
  REGION 1..8: note = Synthetic
LQSSSLRT

SEQ ID NO: 209 - DNA, 360 bp, synthetic construct
  misc_feature 1..360: note = Synthetic
  source 1..360: mol_type = other DNA
caggtgcagctggtggagtctgggggaggcttggtcaagcctggagggtccctgagactctcctgtgcagcctctggattcaccttcagtgactactacatgaactggatccgccaggctccagggaaggggctggagtggatttcatacattagtagtagtggtagtaccacatactacgcagactctgtgaagggccgattcaccatctccagggacaacgccaagaactcactgtttctgcaaatgaacagcctgagaggcgaggacacggccgtgtattattgtgcgagagatgggagatacaacaccgtcgccggggactactggggccagggaaccacggtcaccgtctcctca

SEQ ID NO: 210 - protein, 120 aa, synthetic construct
  REGION 1..120: note = Synthetic
QVQLVESGGGLVKPGGSLRLSCAASGFTFSDYYMNWIRQAPGKGLEWISYISSSGSTTYYADSVKGRFTISRDNAKNSLFLQMNSLRGEDTAVYYCARDGRYNTVAGDYWGQGTTVTVSS

SEQ ID NO: 211 - DNA, 24 bp, synthetic construct
  misc_feature 1..24: note = Synthetic
  source 1..24: mol_type = other DNA
ggattcaccttcagtgactactac

SEQ ID NO: 212 - protein, 8 aa, synthetic construct
  REGION 1..8: note = Synthetic
GFTFSDYY

SEQ ID NO: 213 - DNA, 24 bp, synthetic construct
  misc_feature 1..24: note = Synthetic
  source 1..24: mol_type = other DNA
attagtagtagtggtagtaccaca

SEQ ID NO: 214 - protein, 8 aa, synthetic construct
  REGION 1..8: note = Synthetic
ISSSGSTT

SEQ ID NO: 215 - DNA, 39 bp, synthetic construct
  misc_feature 1..39: note = Synthetic
  source 1..39: mol_type = other DNA
gcgagagatgggagatacaacaccgtcgccggggactac

SEQ ID NO: 216 - protein, 13 aa, synthetic construct
  REGION 1..13: note = Synthetic
ARDGRYNTVAGDY

SEQ ID NO: 217 - DNA, 321 bp, synthetic construct
  misc_feature 1..321: note = Synthetic
  source 1..321: mol_type = other DNA
gaaattgtgatgacgcagtctccagactttcagtctgtggctccaaaggagaaagtcaccatcacctgccgggccagtcagaacattggtggtagcttacactggtaccagcagaaaccagatcagtctccaaagctcctcatcaagtatgcttcccagtccttctcaggggtcccctcgaggttcagtggcagtggatctgggacagatttcaccctcaccatcaatagcctggaagctgaagatgctgcaacgtattactgtcttcagagttacactttacggacgttcggccaagggaccaaggtggagatcaaacga

SEQ ID NO: 218 - protein, 107 aa, synthetic construct
  REGION 1..107: note = Synthetic
EIVMTQSPDFQSVAPKEKVTITCRASQNIGGSLHWYQQKPDQSPKLLIKYASQSFSGVPSRFSGSGSGTDFTLTINSLEAEDAATYYCLQSYTLRTFGQGTKVEIKR

SEQ ID NO: 219 - DNA, 18 bp, synthetic construct
  misc_feature 1..18: note = Synthetic
  source 1..18: mol_type = other DNA
cagaacattggtggtagc

SEQ ID NO: 220 - protein, 6 aa, synthetic construct
  REGION 1..6: note = Synthetic
QNIGGS

SEQ ID NO: 221-222 - skipped (2 entries)

SEQ ID NO: 223 - DNA, 24 bp, synthetic construct
  misc_feature 1..24: note = Synthetic
  source 1..24: mol_type = other DNA
cttcagagttacactttacggacg

SEQ ID NO: 224 - protein, 8 aa, synthetic construct
  REGION 1..8: note = Synthetic
LQSYTLRT

SEQ ID NO: 225 - DNA, 360 bp, synthetic construct
  misc_feature 1..360: note = Synthetic
  source 1..360: mol_type = other DNA
gaggtgcagctggtggagtctgggggaggcttggtcaagcctggagggtccctgagactctcctgtgcagcctctggattcaccttcagtgactactacatgaactggatccgccaggctccagggaaggggctggagtgggtttcatatattagtagtagtggcagcagtatttattacgcagactctgtgaagggccgattcaccatctccagggacaacgccaagaactcactgtatctgctaatgaacagcctgagagccgaggacacggccgtgtattactgtgcgagagatgggaagtataacagttcgccgggggactactggggccagggaaccctggtcaccgtctcctca

SEQ ID NO: 226 - protein, 120 aa, synthetic construct
  REGION 1..120: note = Synthetic
EVQLVESGGGLVKPGGSLRLSCAASGFTFSDYYMNWIRQAPGKGLEWVSYISSSGSSIYYADSVKGRFTISRDNAKNSLYLLMNSLRAEDTAVYYCARDGKYNSSPGDYWGQGTLVTVSS

SEQ ID NO: 227 - DNA, 24 bp, synthetic construct
  misc_feature 1..24: note = Synthetic
  source 1..24: mol_type = other DNA
ggattcaccttcagtgactactac

SEQ ID NO: 228 - protein, 8 aa, synthetic construct
  REGION 1..8: note = Synthetic
GFTFSDYY

SEQ ID NO: 229 - DNA, 24 bp, synthetic construct
  misc_feature 1..24: note = Synthetic
  source 1..24: mol_type = other DNA
attagtagtagtggcagcagtatt

SEQ ID NO: 230 - protein, 8 aa, synthetic construct
  REGION 1..8: note = Synthetic
ISSSGSSI

SEQ ID NO: 231 - DNA, 39 bp, synthetic construct
  misc_feature 1..39: note = Synthetic
  source 1..39: mol_type = other DNA
gcgagagatgggaagtataacagttcgccgggggactac

SEQ ID NO: 232 - protein, 13 aa, synthetic construct
  REGION 1..13: note = Synthetic
ARDGKYNSSPGDY

SEQ ID NO: 233 - DNA, 324 bp, synthetic construct
  misc_feature 1..324: note = Synthetic
  source 1..324: mol_type = other DNA
gacatccagatgacccagtctccatcctcactgtctgcatctgtaggagacagagtcaccatcgcttgtcgggcgagtcagggcattagcaattatttagcctggtttcagcagaaaccagggaaagcccctaagtccctgatctatgctgcatccagtttgcaaagtggggtcccatcaaagttcagcggcagtggatctgggacagatttcactctcaccatcagcagcctgcagcctgaagattttgcaacttattactgccaacagtataacagttacccgctcactttcggcggagggaccaaggtggaaatcaaacga

SEQ ID NO: 234 - protein, 108 aa, synthetic construct
  REGION 1..108: note = Synthetic
DIQMTQSPSSLSASVGDRVTIACRASQGISNYLAWFQQKPGKAPKSLIYAASSLQSGVPSKFSGSGSGTDFTLTISSLQPEDFATYYCQQYNSYPLTFGGGTKVEIKR

SEQ ID NO: 235 - DNA, 18 bp, synthetic construct
  misc_feature 1..18: note = Synthetic
  source 1..18: mol_type = other DNA
cagggcattagcaattat

SEQ ID NO: 236 - protein, 6 aa, synthetic construct
  REGION 1..6: note = Synthetic
QGISNY

SEQ ID NO: 237-238 - skipped (2 entries)

SEQ ID NO: 239 - DNA, 27 bp, synthetic construct
  misc_feature 1..27: note = Synthetic
  source 1..27: mol_type = other DNA
caacagtataacagttacccgctcact

SEQ ID NO: 240 - protein, 9 aa, synthetic construct
  REGION 1..9: note = Synthetic
QQYNSYPLT

SEQ ID NO: 241 - DNA, 360 bp, synthetic construct
  misc_feature 1..360: note = Synthetic
  source 1..360: mol_type = other DNA
gaggtgcagctggtggagtctgggggaggcttggtcaagcctggagggtccctgagactctcctgtgcagcctctggattcaccttcagtgactactacatgaactggatccgccaggctccagggaaggggctggagtgggtttcatatattagtagtagtggcagtagtatttattacgcagactctgtgaagggccgattcaccatctccagggacaacgccaagaactcactgtatctgctaatgaacagcctgagagccgaggacacggccgtgtattactgtgcgagagatgggaagtataacagctcgccgggggactactggggccagggaaccctggtcactgtctcctca

SEQ ID NO: 242 - protein, 120 aa, synthetic construct; identical to SEQ ID NO: 226
  REGION 1..120: note = Synthetic

SEQ ID NO: 243 - DNA, 24 bp, synthetic construct
  misc_feature 1..24: note = Synthetic
  source 1..24: mol_type = other DNA
ggattcaccttcagtgactactac

SEQ ID NO: 244 - protein, 8 aa, synthetic construct
  REGION 1..8: note = Synthetic
GFTFSDYY

SEQ ID NO: 245 - DNA, 24 bp, synthetic construct
  misc_feature 1..24: note = Synthetic
  source 1..24: mol_type = other DNA
attagtagtagtggcagtagtatt

SEQ ID NO: 246 - protein, 8 aa, synthetic construct
  REGION 1..8: note = Synthetic
ISSSGSSI

SEQ ID NO: 247 - DNA, 39 bp, synthetic construct
  misc_feature 1..39: note = Synthetic
  source 1..39: mol_type = other DNA
gcgagagatgggaagtataacagctcgccgggggactac

SEQ ID NO: 248 - protein, 13 aa, synthetic construct
  REGION 1..13: note = Synthetic
ARDGKYNSSPGDY

SEQ ID NO: 249 - DNA, 318 bp, synthetic construct
  misc_feature 1..318: note = Synthetic
  source 1..318: mol_type = other DNA
gaaattgtgctgactcagtctccagactttcagtctgtgactccaaaggagaaagtcaccatcacctgccgggccagtcagagcattggtggtagcttacactggtaccagcagaaaccagatcagtctccaaagctcctcatcaagtatgcttcccagtccttctcaggggtcccctcgaggttcagtggcagtggatctgggacagatttcaccctcaccatcaatagcctggaagctgaagatgctgcaacgtattactgtcttcagagtagtagtttacggacgttcggccaagggaccaaggtggaaatcaaa

SEQ ID NO: 250 - protein, 106 aa, synthetic construct
  REGION 1..106: note = Synthetic
EIVLTQSPDFQSVTPKEKVTITCRASQSIGGSLHWYQQKPDQSPKLLIKYASQSFSGVPSRFSGSGSGTDFTLTINSLEAEDAATYYCLQSSSLRTFGQGTKVEIK

SEQ ID NO: 251 - DNA, 18 bp, synthetic construct
  misc_feature 1..18: note = Synthetic
  source 1..18: mol_type = other DNA
cagagcattggtggtagc

SEQ ID NO: 252 - protein, 6 aa, synthetic construct
  REGION 1..6: note = Synthetic
QSIGGS

SEQ ID NO: 253-254 - skipped (2 entries)

SEQ ID NO: 255 - DNA, 24 bp, synthetic construct
  misc_feature 1..24: note = Synthetic
  source 1..24: mol_type = other DNA
cttcagagtagtagtttacggacg

SEQ ID NO: 256 - protein, 8 aa, synthetic construct
  REGION 1..8: note = Synthetic
LQSSSLRT

SEQ ID NO: 257 - DNA, 363 bp, synthetic construct
  misc_feature 1..363: note = Synthetic
  source 1..363: mol_type = other DNA
gaggtgcagctggtggagtctgggggaggcttggtcaagcctggagggtccctgagactctcctgtgcagcctctggattcaccttcagtgactactacatgaactggatccgccaggctccagggaaggggctggagtgggtttcatacattagtagtagtggtaattccatatactacgcagactctgtgaagggccgattcaccatctccagggacaacgccaagaactcactgtttctgcagatgagcagcctgagagccgaggacacggccgtgtattactgtgcgagagatgggaggtataacgaccgtcgccgggggtactactggggccagggaaccctggtcaccgtctcctca

SEQ ID NO: 258 - protein, 121 aa, synthetic construct
  REGION 1..121: note = Synthetic
EVQLVESGGGLVKPGGSLRLSCAASGFTFSDYYMNWIRQAPGKGLEWVSYISSSGNSIYYADSVKGRFTISRDNAKNSLFLQMSSLRAEDTAVYYCARDGRYNDRRRGYYWGQGTLVTVSS

SEQ ID NO: 259 - DNA, 24 bp, synthetic construct
  misc_feature 1..24: note = Synthetic
  source 1..24: mol_type = other DNA
ggattcaccttcagtgactactac

SEQ ID NO: 260 - protein, 8 aa, synthetic construct
  REGION 1..8: note = Synthetic
GFTFSDYY

SEQ ID NO: 261 - DNA, 24 bp, synthetic construct
  misc_feature 1..24: note = Synthetic
  source 1..24: mol_type = other DNA
attagtagtagtggtaattccata

SEQ ID NO: 262 - protein, 8 aa, synthetic construct
  REGION 1..8: note = Synthetic
ISSSGNSI

SEQ ID NO: 263 - DNA, 42 bp, synthetic construct
  misc_feature 1..42: note = Synthetic
  source 1..42: mol_type = other DNA
gcgagagatgggaggtataacgaccgtcgccgggggtactac

SEQ ID NO: 264 - protein, 14 aa, synthetic construct
  REGION 1..14: note = Synthetic
ARDGRYNDRRRGYY

SEQ ID NO: 265 - DNA, 321 bp, synthetic construct
  misc_feature 1..321: note = Synthetic
  source 1..321: mol_type = other DNA
gaaattgtgatgacgcagtctccagactttcagtctgtgactccaaaggagaaagtcaccatcacctgccgggccagtcagagcattggtagtagcttacactggtaccagcagaaaccagatcagtctccaaaactcctcatcaagtatgcttcccagtccttctcaggggtcccctcgaggttcagtggcagtggatctgggacagatttcaccctcaccatcaatagcctggaagctgaagatgctgcaacgtattactgtcttcagagtagtagtttacggacgttcggccaagggaccaaggtggagatcaaacga

SEQ ID NO: 266 - protein, 107 aa, synthetic construct
  REGION 1..107: note = Synthetic
EIVMTQSPDFQSVTPKEKVTITCRASQSIGSSLHWYQQKPDQSPKLLIKYASQSFSGVPSRFSGSGSGTDFTLTINSLEAEDAATYYCLQSSSLRTFGQGTKVEIKR

SEQ ID NO: 267 - DNA, 18 bp, synthetic construct
  misc_feature 1..18: note = Synthetic
  source 1..18: mol_type = other DNA
cagagcattggtagtagc

SEQ ID NO: 268 - protein, 6 aa, synthetic construct
  REGION 1..6: note = Synthetic
QSIGSS

SEQ ID NO: 269-270 - skipped (2 entries)

SEQ ID NO: 271 - DNA, 24 bp, synthetic construct
  misc_feature 1..24: note = Synthetic
  source 1..24: mol_type = other DNA
cttcagagtagtagtttacggacg

SEQ ID NO: 272 - protein, 8 aa, synthetic construct
  REGION 1..8: note = Synthetic
LQSSSLRT

SEQ ID NO: 273 - DNA, 360 bp, synthetic construct
  misc_feature 1..360: note = Synthetic
  source 1..360: mol_type = other DNA
gaggtgcagctggtggagtctgggggaggcttggtcaagcctggagggtccctgagactctcctgtgcagcctctggattcaccttcagtgactactacatgaactggatccgccaggctccagggaaggggctggagtggatttcatatcttagtagtagtggtagtgccacatactacgcagactctgtgaagggccgattcaccatctccagggacaacgccaagaactcactgtatctgcaaatgaacagcctgagagccgaggacacggccgtgtattattgtgcgagagatgggaagtacaacaccgtcgccggggactactggggccagggaaccacggtcaccgtctcctca

SEQ ID NO: 274 - protein, 120 aa, synthetic construct
  REGION 1..120: note = Synthetic
EVQLVESGGGLVKPGGSLRLSCAASGFTFSDYYMNWIRQAPGKGLEWISYLSSSGSATYYADSVKGRFTISRDNAKNSLYLQMNSLRAEDTAVYYCARDGKYNTVAGDYWGQGTTVTVSS

SEQ ID NO: 275 - DNA, 24 bp, synthetic construct
  misc_feature 1..24: note = Synthetic
  source 1..24: mol_type = other DNA
ggattcaccttcagtgactactac

SEQ ID NO: 276 - protein, 8 aa, synthetic construct
  REGION 1..8: note = Synthetic
GFTFSDYY

SEQ ID NO: 277 - DNA, 24 bp, synthetic construct
  misc_feature 1..24: note = Synthetic
  source 1..24: mol_type = other DNA
cttagtagtagtggtagtgccaca

SEQ ID NO: 278 - protein, 8 aa, synthetic construct
  REGION 1..8: note = Synthetic
LSSSGSAT

SEQ ID NO: 279 - DNA, 39 bp, synthetic construct
  misc_feature 1..39: note = Synthetic
  source 1..39: mol_type = other DNA
gcgagagatgggaagtacaacaccgtcgccggggactac

SEQ ID NO: 280 - protein, 13 aa, synthetic construct
  REGION 1..13: note = Synthetic
ARDGKYNTVAGDY

SEQ ID NO: 281 - DNA, 324 bp, synthetic construct
  misc_feature 1..324: note = Synthetic
  source 1..324: mol_type = other DNA
gacatccagttgacccagtctccatcctccctgtctgcatctgtaggagacagagtcaccatcacttgccgggcaagtcagggcattagaaatgatttaggctggtatcagcagaaaccagggaaagcccctaagcgcctgatctatgctgcatccagtttacaaagtggggtcccatcaaggttcagcggcagtggatctgggacagaattcactctcacaatcagcagcctgcagcctgaagattttgcaacttattactgtctacaacataatagttacccgtacacttttggccaggggaccaaggtagagatcaaacga

SEQ ID NO: 282 - protein, 108 aa, synthetic construct
  REGION 1..108: note = Synthetic
DIQLTQSPSSLSASVGDRVTITCRASQGIRNDLGWYQQKPGKAPKRLIYAASSLQSGVPSRFSGSGSGTEFTLTISSLQPEDFATYYCLQHNSYPYTFGQGTKVEIKR

SEQ ID NO: 283 - DNA, 18 bp, synthetic construct
  misc_feature 1..18: note = Synthetic
  source 1..18: mol_type = other DNA
cagggcattagaaatgat

SEQ ID NO: 284 - protein, 6 aa, synthetic construct
  REGION 1..6: note = Synthetic
QGIRND

SEQ ID NO: 285-286 - skipped (2 entries)

SEQ ID NO: 287 - DNA, 27 bp, synthetic construct
  misc_feature 1..27: note = Synthetic
  source 1..27: mol_type = other DNA
ctacaacataatagttacccgtacact

SEQ ID NO: 288 - protein, 9 aa, synthetic construct
  REGION 1..9: note = Synthetic
LQHNSYPYT

SEQ ID NO: 289 - DNA, 360 bp, synthetic construct
  misc_feature 1..360: note = Synthetic
  source 1..360: mol_type = other DNA
gaggtgcagctggtggagtctgggggaggcttggtcaagcctggagggtccctgagactctcctgtgcagcctctggattcaccttcagtgactactacatgaactggatccgccaggctccagggaaggggctggagtggatttcatacattagtagtagtgatgataccacatactacgcagactctgtgaagggccgattcaccatatccagggacaacgccaagaactcactgtatctgcaaatgaacagcctgagagccgaggacacggccgtgtattattgtgcgagagatgggaagtacaacaccgtcgccggggaccactggggccagggaaccctggtcaccgtctcctca

SEQ ID NO: 290 - protein, 120 aa, synthetic construct
  REGION 1..120: note = Synthetic
EVQLVESGGGLVKPGGSLRLSCAASGFTFSDYYMNWIRQAPGKGLEWISYISSSDDTTYYADSVKGRFTISRDNAKNSLYLQMNSLRAEDTAVYYCARDGKYNTVAGDHWGQGTLVTVSS

SEQ ID NO: 291 - DNA, 24 bp, synthetic construct
  misc_feature 1..24: note = Synthetic
  source 1..24: mol_type = other DNA
ggattcaccttcagtgactactac

SEQ ID NO: 292 - protein, 8 aa, synthetic construct
  REGION 1..8: note = Synthetic
GFTFSDYY

SEQ ID NO: 293 - DNA, 24 bp, synthetic construct
  misc_feature 1..24: note = Synthetic
  source 1..24: mol_type = other DNA
attagtagtagtgatgataccaca

SEQ ID NO: 294 - protein, 8 aa, synthetic construct
  REGION 1..8: note = Synthetic
ISSSDDTT

SEQ ID NO: 295 - DNA, 39 bp, synthetic construct
  misc_feature 1..39: note = Synthetic
  source 1..39: mol_type = other DNA
gcgagagatgggaagtacaacaccgtcgccggggaccac

SEQ ID NO: 296 - protein, 13 aa, synthetic construct
  REGION 1..13: note = Synthetic
ARDGKYNTVAGDH

SEQ ID NO: 297 - DNA, 321 bp, synthetic construct
  misc_feature 1..321: note = Synthetic
  source 1..321: mol_type = other DNA
gaaattgtgatgacacagtctccagactttcagtctgtggctccaaaggagaaagtcaccatcacctgccgggccagtcagaacattggtagtagcttacactggtaccagcagaaaccagatcagtctccaaagctcctcatcaagtatgcttcccagtccttctcaggggtcccctcgaggttcagtggcagtggatctgggacagatttcaccctcaccatcaatagcctggaagctgaagatgctgcaacgtattactgtcttcagagttatactttaaggacgttcggccaagggaccaaggtggagatcaaacga

SEQ ID NO: 298 - protein, 107 aa, synthetic construct
  REGION 1..107: note = Synthetic
EIVMTQSPDFQSVAPKEKVTITCRASQNIGSSLHWYQQKPDQSPKLLIKYASQSFSGVPSRFSGSGSGTDFTLTINSLEAEDAATYYCLQSYTLRTFGQGTKVEIKR

SEQ ID NO: 299 - DNA, 18 bp, synthetic construct
  misc_feature 1..18: note = Synthetic
  source 1..18: mol_type = other DNA
cagaacattggtagtagc

SEQ ID NO: 300 - protein, 6 aa, synthetic construct
  REGION 1..6: note = Synthetic
QNIGSS

SEQ ID NO: 301-302 - skipped (2 entries)

SEQ ID NO: 303 - DNA, 24 bp, synthetic construct
  misc_feature 1..24: note = Synthetic
  source 1..24: mol_type = other DNA
cttcagagttatactttaaggacg

SEQ ID NO: 304 - protein, 8 aa, synthetic construct
  REGION 1..8: note = Synthetic
LQSYTLRT

SEQ ID NO: 305 - DNA, 345 bp, synthetic construct
  misc_feature 1..345: note = Synthetic
  source 1..345: mol_type = other DNA
gaggtgcagctggtggagtctgggggaggcttggtacagcctggggggtccctgagactctcctgtgcagcctctggattcacctttagcagttatgccatgagctgggtccgccaggctccagggaaggggctggagtgggtctcagctattagtggtcgtggttataacgcagactacgcagactccgtgaagggccggttcaccatctccagggacaattccaagaacacgctgtatctgcaaatgaacagcctgagagccgaagacacggccgtatattactgtgcgaaattggaatactttgactactggggccagggaaccctggtcactgtctcctca

SEQ ID NO: 306 - protein, 115 aa, synthetic construct
  REGION 1..115: note = Synthetic
EVQLVESGGGLVQPGGSLRLSCAASGFTFSSYAMSWVRQAPGKGLEWVSAISGRGYNADYADSVKGRFTISRDNSKNTLYLQMNSLRAEDTAVYYCAKLEYFDYWGQGTLVTVSS

SEQ ID NO: 307 - DNA, 24 bp, synthetic construct
  misc_feature 1..24: note = Synthetic
  source 1..24: mol_type = other DNA
ggattcacctttagcagttatgcc

SEQ ID NO: 308 - protein, 8 aa, synthetic construct
  REGION 1..8: note = Synthetic
GFTFSSYA

SEQ ID NO: 309 - DNA, 24 bp, synthetic construct
  misc_feature 1..24: note = Synthetic
  source 1..24: mol_type = other DNA
attagtggtcgtggttataacgca

SEQ ID NO: 310 - protein, 8 aa, synthetic construct
  REGION 1..8: note = Synthetic
ISGRGYNA

SEQ ID NO: 311 - DNA, 24 bp, synthetic construct
  misc_feature 1..24: note = Synthetic
  source 1..24: mol_type = other DNA
gcgaaattggaatactttgactac

SEQ ID NO: 312 - protein, 8 aa, synthetic construct
  REGION 1..8: note = Synthetic
AKLEYFDY

SEQ ID NO: 313 - DNA, 321 bp, synthetic construct
  misc_feature 1..321: note = Synthetic
  source 1..321: mol_type = other DNA
gacatccagatgacccagtctccttccaccctgtctgcatctgtaggagacagagtcaccatcacttgccgggccagtcagagtattagtagctggttggcctggtatcagcagaaaccagggaaagcccctaagctcctgatctataaggcgtctagtttagaaagtggggtcccatcaaggttcagcggcagtggatctgggacagatttcactctcaccatcagcagcctgaggcctgaagattttgcaacttattactgccaacagtataatagttaccctctgactttcggcggagggaccaaggtggagatcaaa

SEQ ID NO: 314 - protein, 107 aa, synthetic construct
  REGION 1..107: note = Synthetic
DIQMTQSPSTLSASVGDRVTITCRASQSISSWLAWYQQKPGKAPKLLIYKASSLESGVPSRFSGSGSGTDFTLTISSLRPEDFATYYCQQYNSYPLTFGGGTKVEIK

SEQ ID NO: 315 - DNA, 18 bp, synthetic construct
  misc_feature 1..18: note = Synthetic
  source 1..18: mol_type = other DNA
cagagtattagtagctgg

SEQ ID NO: 316 - protein, 6 aa, synthetic construct
  REGION 1..6: note = Synthetic
QSISSW

SEQ ID NO: 317-318 - skipped (2 entries)

SEQ ID NO: 319 - DNA, 27 bp, synthetic construct
  misc_feature 1..27: note = Synthetic
  source 1..27: mol_type = other DNA
caacagtataatagttaccctctgact

SEQ ID NO: 320 - protein, 9 aa, synthetic construct
  REGION 1..9: note = Synthetic
QQYNSYPLT

SEQ ID NO: 321 - DNA, 345 bp, synthetic construct
  misc_feature 1..345: note = Synthetic
  source 1..345: mol_type = other DNA
gaggtgcagctggtggagtctgggggaggcttggtacagcctggggggtccctgagactctcctgtgcagcctctggattcacctttagcacctatgccatgcactgggtccgccaggctccagggaaggggctggagtgggtctcaagtattagtggtcgtggtcgtaactcagaccacgcagactccgtgaagggccggttcaccatctccagagacaattccaagaacacgctctatctacaaatgaacagcctgagagccgaggacacggccgtatattactgtgcgaggaccgaatacttccaccactggggccagggcaccctggtcaccgtctcctca

SEQ ID NO: 322 - protein, 115 aa, synthetic construct
  REGION 1..115: note = Synthetic
EVQLVESGGGLVQPGGSLRLSCAASGFTFSTYAMHWVRQAPGKGLEWVSSISGRGRNSDHADSVKGRFTISRDNSKNTLYLQMNSLRAEDTAVYYCARTEYFHHWGQGTLVTVSS

SEQ ID NO: 323 - DNA, 24 bp, synthetic construct
  misc_feature 1..24: note = Synthetic
  source 1..24: mol_type = other DNA
ggattcacctttagcacctatgcc

SEQ ID NO: 324 - protein, 8 aa, synthetic construct
  REGION 1..8: note = Synthetic
GFTFSTYA

SEQ ID NO: 325 - DNA, 24 bp, synthetic construct
  misc_feature 1..24: note = Synthetic
  source 1..24: mol_type = other DNA
attagtggtcgtggtcgtaactca

SEQ ID NO: 326 - protein, 8 aa, synthetic construct
  REGION 1..8: note = Synthetic
ISGRGRNS

SEQ ID NO: 327 - DNA, 24 bp, synthetic construct
  misc_feature 1..24: note = Synthetic
  source 1..24: mol_type = other DNA
gcgaggaccgaatacttccaccac

SEQ ID NO: 328 - protein, 8 aa, synthetic construct
  REGION 1..8: note = Synthetic
ARTEYFHH

SEQ ID NO: 329 - DNA, 321 bp, synthetic construct
  misc_feature 1..321: note = Synthetic
  source 1..321: mol_type = other DNA
gacatccagatgacccagtctccatcctcactgtctgcatctgtaggagacagaatcaccatcacttgtcgggcgagtcaggacattaacaattatttagcctggtttcagcagaaaccaggaaaagcccctaagtccctgatctatggtgcatccagcttgcaaagtggggtcccatcaaagttcagcggcagtggatctgggacagatttcactctcaccatcagcagcctgcagcctgaagattttgcaacttattactgccaacaatatagttcttacccattcactttcggccctgggaccaaagtggatatcaaa

SEQ ID NO: 330 - protein, 107 aa, synthetic construct
  REGION 1..107: note = Synthetic
DIQMTQSPSSLSASVGDRITITCRASQDINNYLAWFQQKPGKAPKSLIYGASSLQSGVPSKFSGSGSGTDFTLTISSLQPEDFATYYCQQYSSYPFTFGPGTKVDIK

SEQ ID NO: 331 - DNA, 18 bp, synthetic construct
  misc_feature 1..18: note = Synthetic
  source 1..18: mol_type = other DNA
caggacattaacaattat

SEQ ID NO: 332 - protein, 6 aa, synthetic construct
  REGION 1..6: note = Synthetic
QDINNY

SEQ ID NO: 333-334 - skipped (2 entries)

SEQ ID NO: 335 - DNA, 27 bp, synthetic construct
  misc_feature 1..27: note = Synthetic
  source 1..27: mol_type = other DNA
caacaatatagttcttacccattcact

SEQ ID NO: 336 - protein, 9 aa, synthetic construct
  REGION 1..9: note = Synthetic
QQYSSYPFT

SEQ ID NO: 337 - DNA, 348 bp, synthetic construct
  misc_feature 1..348: note = Synthetic
  source 1..348: mol_type = other DNA
gaggtgcagctggtggagtctgggggaggcttggtccagcctggggggtccctgagactctcctgtgcagcctctggattcatctttagtacctattggatgaactgggtccgccaggctccagggaaggggctggagtgggtggccaacgtgaaccatgatggaagtgaggaatactatgtggactctgtgaagggccgattcaccatctccagagacaacgcccagaattcactgtatctgcaaatggaccgcctgagagccgaggacacggctatgtatttctgtgcgcgaagagccgggctttttgactcctggggccagggaaccctggtcactgtctcctca

SEQ ID NO: 338 - protein, 116 aa, synthetic construct
  REGION 1..116: note = Synthetic
EVQLVESGGGLVQPGGSLRLSCAASGFIFSTYWMNWVRQAPGKGLEWVANVNHDGSEEYYVDSVKGRFTISRDNAQNSLYLQMDRLRAEDTAMYFCARRAGLFDSWGQGTLVTVSS

SEQ ID NO: 339 - DNA, 24 bp, synthetic construct
  misc_feature 1..24: note = Synthetic
  source 1..24: mol_type = other DNA
ggattcatctttagtacctattgg

SEQ ID NO: 340 - protein, 8 aa, synthetic construct
  REGION 1..8: note = Synthetic
GFIFSTYW

SEQ ID NO: 341 - DNA, 24 bp, synthetic construct
  misc_feature 1..24: note = Synthetic
  source 1..24: mol_type = other DNA
gtgaaccatgatggaagtgaggaa

SEQ ID NO: 342 - protein, 8 aa, synthetic construct
  REGION 1..8: note = Synthetic
VNHDGSEE

SEQ ID NO: 343 - DNA, 27 bp, synthetic construct
  misc_feature 1..27: note = Synthetic
  source 1..27: mol_type = other DNA
gcgcgaagagccgggctttttgactcc

SEQ ID NO: 344 - protein, 9 aa, synthetic construct
  REGION 1..9: note = Synthetic
ARRAGLFDS

SEQ ID NO: 345 - DNA, 321 bp, synthetic construct
  misc_feature 1..321: note = Synthetic
  source 1..321: mol_type = other DNA
gacatccagatgacccagtctccatcttccgtgtctgcatctgtaggagacagagtcaccatcacttgtcgggcgagtcaggatattgacaactggttagcctggtatcagcagaaaccagggaaagcccctaaactcctgatctttacttcatccactttgcaaagtggggtcccatcaaggttcagcggcattggatctggaacagatttcactctcaccatcagcagcctacagcctgaagattttgcaacttactattgtcaacaggctaacagtttcccgtggacgttcggccaagggaccaaggtggagatcaaa

SEQ ID NO: 346 - protein, 107 aa, synthetic construct
  REGION 1..107: note = Synthetic
DIQMTQSPSSVSASVGDRVTITCRASQDIDNWLAWYQQKPGKAPKLLIFTSSTLQSGVPSRFSGIGSGTDFTLTISSLQPEDFATYYCQQANSFPWTFGQGTKVEIK

SEQ ID NO: 347 - DNA, 18 bp, synthetic construct
  misc_feature 1..18: note = Synthetic
  source 1..18: mol_type = other DNA
caggatattgacaactgg

SEQ ID NO: 348 - protein, 6 aa, synthetic construct
  REGION 1..6: note = Synthetic
QDIDNW

SEQ ID NO: 349-350 - skipped (2 entries)

SEQ ID NO: 351 - DNA, 27 bp, synthetic construct
  misc_feature 1..27: note = Synthetic
  source 1..27: mol_type = other DNA
caacaggctaacagtttcccgtggacg

SEQ ID NO: 352 - protein, 9 aa, synthetic construct
  REGION 1..9: note = Synthetic
QQANSFPWT

SEQ ID NO: 353 - DNA, 375 bp, synthetic construct
  misc_feature 1..375: note = Synthetic
  source 1..375: mol_type = other DNA
caggtgcagctggtggagtctgggggaggcgtggtcctgcctgggaggtccctgagactctcctgtgcagcgtctggattcacctttagtagttatctcatgtattgggtccgccaggctccaggcaaggggctggagtgggtggcagttatatggtatgatggaagtaataaattctatggagactccgtgaagggccgattcaccatctccagagacaattccaagaacacgttgtatctgcaaatgaacagcctgagagccgaggacacggctgtgtattactgtgcgagagataatgggaatagtggttacgaggacagctggaatgcttttgatatatggggccaagggacaatggtcaccgtctcttca

SEQ ID NO: 354 - protein, 125 aa, synthetic construct
  REGION 1..125: note = Synthetic
QVQLVESGGGVVLPGRSLRLSCAASGFTFSSYLMYWVRQAPGKGLEWVAVIWYDGSNKFYGDSVKGRFTISRDNSKNTLYLQMNSLRAEDTAVYYCARDNGNSGYEDSWNAFDIWGQGTMVTVSS

SEQ ID NO: 355 - DNA, 24 bp, synthetic construct
  misc_feature 1..24: note = Synthetic
  source 1..24: mol_type = other DNA
ggattcacctttagtagttatctc

SEQ ID NO: 356 - protein, 8 aa, synthetic construct
  REGION 1..8: note = Synthetic
GFTFSSYL

SEQ ID NO: 357 - DNA, 24 bp, synthetic construct
  misc_feature 1..24: note = Synthetic
  source 1..24: mol_type = other DNA
atatggtatgatggaagtaataaa

SEQ ID NO: 358 - protein, 8 aa, synthetic construct
  REGION 1..8: note = Synthetic
IWYDGSNK

SEQ ID NO: 359 - DNA, 54 bp, synthetic construct
  misc_feature 1..54: note = Synthetic
  source 1..54: mol_type = other DNA
gcgagagataatgggaatagtggttacgaggacagctggaatgcttttgatata

SEQ ID NO: 360 - protein, 18 aa, synthetic construct
  REGION 1..18: note = Synthetic
ARDNGNSGYEDSWNAFDI

SEQ ID NO: 361 - DNA, 321 bp, synthetic construct
  misc_feature 1..321: note = Synthetic
  source 1..321: mol_type = other DNA
gacatccagatgacccagtctccatcctcactgtctgcatctgtaggagacagagtcaccatcacttgtcgggcgagtcaggacatttacaattatttagcctggtttcagcagaaaccagggaaagcccctaagtccctgatctatgctgcatccagtttgcaaactggggtcccatcacagttcagcggcagtggatctgggacagatttcactctcaccatcagcagcctccagcctgaagattttgcaacttattactgccaacagtataataattacccattcactttcggccctgggaccaaagtggatatcaaa

SEQ ID NO: 362 - protein, 107 aa, synthetic construct
  REGION 1..107: note = Synthetic
DIQMTQSPSSLSASVGDRVTITCRASQDIYNYLAWFQQKPGKAPKSLIYAASSLQTGVPSQFSGSGSGTDFTLTISSLQPEDFATYYCQQYNNYPFTFGPGTKVDIK

SEQ ID NO: 363 - DNA, 18 bp, synthetic construct
  misc_feature 1..18: note = Synthetic
  source 1..18: mol_type = other DNA
caggacatttacaattat

SEQ ID NO: 364 - protein, 6 aa, synthetic construct
  REGION 1..6: note = Synthetic
QDIYNY

SEQ ID NO: 365-366 - skipped (2 entries)

SEQ ID NO: 367 - DNA, 27 bp, synthetic construct
  misc_feature 1..27: note = Synthetic
  source 1..27: mol_type = other DNA
caacagtataataattacccattcact

SEQ ID NO: 368 - protein, 9 aa, synthetic construct
  REGION 1..9: note = Synthetic
QQYNNYPFT

SEQ ID NO: 369 - DNA, 360 bp, synthetic construct
  misc_feature 1..360: note = Synthetic
  source 1..360: mol_type = other DNA
gaggtgcagctggtggagtctgggggaggcttggcacagcctggggggtccctgagactctcctgtgcagcctctggattcacctttaacaactatgccatgacctgggtccgccaggctccagggaagggtctggactgggtctcagctattagtgatagtggtcgtagcacattctccgcagactccgtgaagggccggttcaccatctccagagacaactccaagaacacgctgtatctgcaaatggacagcctgagagccgaggacacggccttatattactgtgcgaaacataggaactggaactatcccgtctttgactactggggccagggaaccctggtcaccgtctcctca

SEQ ID NO: 370 - protein, 120 aa, synthetic construct
  REGION 1..120: note = Synthetic
EVQLVESGGGLAQPGGSLRLSCAASGFTFNNYAMTWVRQAPGKGLDWVSAISDSGRSTFSADSVKGRFTISRDNSKNTLYLQMDSLRAEDTALYYCAKHRNWNYPVFDYWGQGTLVTVSS

SEQ ID NO: 371 - DNA, 24 bp, synthetic construct
  misc_feature 1..24: note = Synthetic
  source 1..24: mol_type = other DNA
ggattcacctttaacaactatgcc

SEQ ID NO: 372 - protein, 8 aa, synthetic construct
  REGION 1..8: note = Synthetic
GFTFNNYA

SEQ ID NO: 373 - DNA, 24 bp, synthetic construct
  misc_feature 1..24: note = Synthetic
  source 1..24: mol_type = other DNA
attagtgatagtggtcgtagcaca

SEQ ID NO: 374 - protein, 8 aa, synthetic construct
  REGION 1..8: note = Synthetic
ISDSGRST

SEQ ID NO: 375 - DNA, 39 bp, synthetic construct
  misc_feature 1..39: note = Synthetic
  source 1..39: mol_type = other DNA
gcgaaacataggaactggaactatcccgtctttgactac

SEQ ID NO: 376 - protein, 13 aa, synthetic construct
  REGION 1..13: note = Synthetic
AKHRNWNYPVFDY

SEQ ID NO: 377 - DNA, 321 bp, synthetic construct
  misc_feature 1..321: note = Synthetic
  source 1..321: mol_type = other DNA
gacatccagttgacccagtctccatccttcctgtctgcatctgtgggagacagagtcaccatcacttgctgggccagtcagggcattagtagttatttagcctggtatcagcaaaaaccagggaaagccccaaagctcctgatctattctgcatccactttacaaagtggggtcccatcaaggttcagcggcagtggatctgggacagaattcactctcacaatcagcagcctgcagcctgaagattttgcaacttattactgtcaacaacttaatagttacccattcactttcggccctgggaccaaagtggatatcaaa

SEQ ID NO: 378 - protein, 107 aa, synthetic construct
  REGION 1..107: note = Synthetic
DIQLTQSPSFLSASVGDRVTITCWASQGISSYLAWYQQKPGKAPKLLIYSASTLQSGVPSRFSGSGSGTEFTLTISSLQPEDFATYYCQQLNSYPFTFGPGTKVDIK

SEQ ID NO: 379 - DNA, 18 bp, synthetic construct
  misc_feature 1..18: note = Synthetic
  source 1..18: mol_type = other DNA
cagggcattagtagttat

SEQ ID NO: 380 - protein, 6 aa, synthetic construct
  REGION 1..6: note = Synthetic
QGISSY

SEQ ID NO: 381-382 - skipped (2 entries)

SEQ ID NO: 383 - DNA, 27 bp, synthetic construct
  misc_feature 1..27: note = Synthetic
  source 1..27: mol_type = other DNA
caacaacttaatagttacccattcact

SEQ ID NO: 384 - protein, 9 aa, synthetic construct
  REGION 1..9: note = Synthetic
QQLNSYPFT

SEQ ID NO: 385 - protein, 190 aa, synthetic construct
  REGION 1..190: note = Synthetic
VKMAETCPIFYDVFFAVANGNELLLDLSLTKVNATEPERTAMKKIQDCYVENGLISRVLDGLVMTTISSSKDCMGEAVQNTVEDLKLNTLGREICPAVKRDVDLFLTGTPDEYVEQVAQYKALPVVLENARILKNCVDAKMTEEDKENALSVLDKIYTSPLCEQKLISEEDLGGEQKLISEEDLHHHHHH

SEQ ID NO: 386-391 - skipped (6 entries)

SEQ ID NO: 392 - protein, 70 aa, synthetic construct
  REGION 1..70: note = Synthetic
EICPAVKRDVDLFLTGTPDEYVEQVAQYKALPVVLENARILKNCVDAKMTEEDKENALSLLDKIYTSPLC

SEQ ID NO: 393 - protein, 92 aa, synthetic construct
  REGION 1..92: note = Synthetic
VKMAETCPIFYDVFFAVANGNELLLDLSLTKVNATEPERTAMKKIQDCYVENGLISRVLDGLVMTTISSSKDCMGEAVQNTVEDLKLNTLGR

SEQ ID NO: 394 - protein, 398 aa, synthetic construct
  REGION 1..398: note = Synthetic
VKMAETCPIFYDVFFAVANGNELLLDLSLTKVNATEPERTAMKKIQDCYVENGLISRVLDGLVMTTISSSKDCMGEAVQNTVEDLKLNTLGREICPAVKRDVDLFLTGTPDEYVEQVAQYKALPVVLENARILKNCVDAKMTEEDKENALSLLDKIYTSPLCLINEPRGPTIKPCPPCKCPAPNLLGGPSVFIFPPKIKDVLMISLSPIVTCVVVDVSEDDPDVQISWFVNNVEVHTAQTQTHREDYNSTLRVVSALPIQHQDWMSGKEFKCKVNNKDLPAPIERTISKPKGSVRAPQVYVLPPPEEEMTKKQVTLTCMVTDFMPEDIYVEWTNNGKTELNYKNTEPVLDSDGSYFMYSKLRVEKKNWVERNSYSCSVVHEGLHNHHTTKSFSRTPGK

SEQ ID NO: 395 - protein, 413 aa, synthetic construct
  REGION 1..413: note = Synthetic
EICPAVKRDVDLFLTGTPDEYVEQVAQYKALPVVLENARILKNCVDAKMTEEDKENALSLLDKIYTSPLCGGGGSGGGGSGGGGSVKMAETCPIFYDVFFAVANGNELLLDLSLTKVNATEPERTAMKKIQDCYVENGLISRVLDGLVMTTISSSKDCMGEAVQNTVEDLKLNTLGRLINEPRGPTIKPCPPCKCPAPNLLGGPSVFIFPPKIKDVLMISLSPIVTCVVVDVSEDDPDVQISWFVNNVEVHTAQTQTHREDYNSTLRVVSALPIQHQDWMSGKEFKCKVNNKDLPAPIERTISKPKGSVRAPQVYVLPPPEEEMTKKQVTLTCMVTDFMPEDIYVEWTNNGKTELNYKNTEPVLDSDGSYFMYSKLRVEKKNWVERNSYSCSVVHEGLHNHHTTKSFSRTPGK

SEQ ID NO: 396 - protein, 199 aa, synthetic construct
  REGION 1..199: note = Synthetic
VKMAETCPIFYDVFFAVANGNELLLDLSLTKVNATEPERTAMKKIQDCYVENGLISRVLDGLVMTTISSSKDCMGEAVQNTVEDLKLNTLGREICPAVKRGVDLFLTGTPDEYVEQVAQYKALPVVLENARILKNCVDAKMTEEDKENALSLLDKIYTSPLCGPGGEQKLISEEDLGGEQKLISEEDLSGHHHHHHSSG

SEQ ID NO: 397 - protein, 214 aa, synthetic construct
  REGION 1..214: note = Synthetic
EICPAVKRDVDLFLTGTPDEYVEQVAQYKALPVVLENARILKNCVDAKMTEEDKENALSLLDKIYTSPLCGGGGSGGGGSGGGGSVKMAETCPIFYDVFFAVANGNELLLDLSLTKVNATEPERTAMKKIQDCYVENGLISRVLDGLVMTTISSSKDCMGEAVQNTVEDLKLNTLGRGPGGEQKLISEEDLGGEQKLISEEDLSGHHHHHHSSG

SEQ ID NO: 398 - protein, 11 aa, synthetic construct
  REGION 1..11: note = Synthetic
VKMAETCPIFY

SEQ ID NO: 399 - protein, 7 aa, synthetic construct
  REGION 1..7: note = Synthetic
ISRVLDG

SEQ ID NO: 400 - protein, 8 aa, synthetic construct
  REGION 1..8: note = Synthetic
ISRVLDGL

SEQ ID NO: 401 - protein, 10 aa, synthetic construct
  REGION 1..10: note = Synthetic
ISRVLDGLVM

SEQ ID NO: 402 - protein, 19 aa, synthetic construct
  REGION 1..19: note = Synthetic
LKLNTLGREICPAVKRGVD

SEQ ID NO: 403 - protein, 20 aa, synthetic construct
  REGION 1..20: note = Synthetic
LKLNTLGREICPAVKRGVDL

SEQ ID NO: 404 - protein, 15 aa, synthetic construct
  REGION 1..15: note = Synthetic
YVEQVAQYKALPVVL

SEQ ID NO: 405 - protein, 11 aa, synthetic construct
  REGION 1..11: note = Synthetic
VAQYKALPVVL

SEQ ID NO: 406 - protein, 14 aa, synthetic construct
  REGION 1..14: note = Synthetic
ENARILKNCVDAKM

SEQ ID NO: 407 - protein, 18 aa, synthetic construct
  REGION 1..18: note = Synthetic
LDKIYTSPLCGPGGEQKL

SEQ ID NO: 408 - protein, 14 aa, synthetic construct
  REGION 1..14: note = Synthetic
ISEEDLSGHHHHHH

SEQ ID NO: 409 - protein, 17 aa, synthetic construct
  REGION 1..17: note = Synthetic
ISEEDLSGHHHHHHSSG

SEQ ID NO: 410 - protein, 14 aa, synthetic construct
  REGION 1..14: note = Synthetic
EDLSGHHHHHHSSG

SEQ ID NO: 411 - protein, 11 aa, synthetic construct
  REGION 1..11: note = Synthetic
VKMAETCPIFY

SEQ ID NO: 412 - protein, 10 aa, synthetic construct
  REGION 1..10: note = Synthetic
FAVANGNELL

SEQ ID NO: 413 - protein, 7 aa, synthetic construct
  REGION 1..7: note = Synthetic
ISRVLDG

SEQ ID NO: 414 - protein, 8 aa, synthetic construct
  REGION 1..8: note = Synthetic
ISRVLDGL

SEQ ID NO: 415 - protein, 10 aa, synthetic construct
  REGION 1..10: note = Synthetic
ISRVLDGLVM

SEQ ID NO: 416 - protein, 19 aa, synthetic construct
  REGION 1..19: note = Synthetic
LKLNTLGREICPAVKRGVD

SEQ ID NO: 417 - protein, 20 aa, synthetic construct
  REGION 1..20: note = Synthetic
LKLNTLGREICPAVKRGVDL

SEQ ID NO: 418 - protein, 15 aa, synthetic construct
  REGION 1..15: note = Synthetic
YVEQVAQYKALPVVL

SEQ ID NO: 419 - protein, 11 aa, synthetic construct
  REGION 1..11: note = Synthetic
VAQYKALPVVL

SEQ ID NO: 420 - protein, 8 aa, synthetic construct
  REGION 1..8: note = Synthetic
YKALPVVL

SEQ ID NO: 421 - protein, 14 aa, synthetic construct
  REGION 1..14: note = Synthetic
ENARILKNCVDAKM

SEQ ID NO: 422 - protein, 18 aa, synthetic construct
  REGION 1..18: note = Synthetic
LDKIYTSPLCGPGGEQKL

SEQ ID NO: 423 - protein, 14 aa, synthetic construct
  REGION 1..14: note = Synthetic
ISEEDLSGHHHHHH

SEQ ID NO: 424 - protein, 17 aa, synthetic construct
  REGION 1..17: note = Synthetic
ISEEDLSGHHHHHHSSG

SEQ ID NO: 425 - protein, 14 aa, synthetic construct
  REGION 1..14: note = Synthetic
EDLSGHHHHHHSSG

SEQ ID NO: 426 - protein, 4 aa, synthetic construct
  REGION 1..4: note = Synthetic
YVEQ

SEQ ID NO: 427 - DNA, 363 bp, synthetic construct
  misc_feature 1..363: note = Synthetic
  source 1..363: mol_type = other DNA
gaggtgcagctggtggagtcgggcccaggactggtgaacccttcggagaccctgtccctcacctgctctgtctctggtggctccatcagcagtgttaattactactggggctggatccgccagtccccagggaagggactggagtggattgggagtatctattatactgggagtaccgactacaacccgtccctcaagaatcgagtcaccatatccgtagacacgtccaagaaccagttctccctgaagcagacttctgtgaccgccgcagacacggctgtctattactgtgcgagacatgtggcactggctggggggcttttgatagtctggggccaggggacaatggtcaccgtctcttca

SEQ ID NO: 428 - protein, 121 aa, synthetic construct
  REGION 1..121: note = Synthetic
EVQLVESGPGLVNPSETLSLTCSVSGGSISSVNYYWGWIRQSPGKGLEWIGSIYYTGSTDYNPSLKNRVTISVDTSKNQFSLKQTSVTAADTAVYYCARHVALAGGLLIVWGQGTMVTVSS

SEQ ID NO: 429 - DNA, 30 bp, synthetic construct; identical to SEQ ID NO: 179
  misc_feature 1..30: note = Synthetic
  source 1..30: mol_type = other DNA

SEQ ID NO: 430 - protein, 10 aa, synthetic construct
  REGION 1..10: note = Synthetic
GGSISSVNYY

SEQ ID NO: 431 - DNA, 21 bp, synthetic construct
  misc_feature 1..21: note = Synthetic
  source 1..21: mol_type = other DNA
atctattatactgggagtacc

SEQ ID NO: 432 - protein, 7 aa, synthetic construct
  REGION 1..7: note = Synthetic
IYYTGST

SEQ ID NO: 433 - DNA, 39 bp, synthetic construct
  misc_feature 1..39: note = Synthetic
  source 1..39: mol_type = other DNA
gcgagacatgtggcactggctggggggcttttgatagtc

SEQ ID NO: 434 - protein, 13 aa, synthetic construct
  REGION 1..13: note = Synthetic
ARHVALAGGLLIV

SEQ ID NO: 435 - DNA, 342 bp, synthetic construct
  misc_feature 1..342: note = Synthetic
  source 1..342: mol_type = other DNA
gacatccagatgacccagtctccagactccctggctgtgtctctgggcgcgagggccaccatcaactgcaagtccagccaaagtgttttattcagctccaacaataagaacttcttagcctggtaccagcagaaaccaggacagcctcctaccctgctcatttcctgggcatctacccgggaatccggggtccctgaccgattcagtgggagcgggtctgggacagatttcactctcaccatcagcagcctgcaggctgaagatgtggcagtttatttctgtcaacaatattataatagtcctccacttttcggccaggggaccaaggtggagatcaaacga

SEQ ID NO: 436 - protein, 114 aa, synthetic construct
  REGION 1..114: note = Synthetic
DIQMTQSPDSLAVSLGARATINCKSSQSVLFSSNNKNFLAWYQQKPGQPPTLLISWASTRESGVPDRFSGSGSGTDFTLTISSLQAEDVAVYFCQQYYNSPPLFGQGTKVEIKR

SEQ ID NO: 437 - DNA, 36 bp, synthetic construct
  misc_feature 1..36: note = Synthetic
  source 1..36: mol_type = other DNA
caaagtgttttattcagctccaacaataagaacttc

SEQ ID NO: 438 - protein, 12 aa, synthetic construct
  REGION 1..12: note = Synthetic
QSVLFSSNNKNF

SEQ ID NO: 439-440 - skipped (2 entries)

SEQ ID NO: 441 - DNA, 27 bp, synthetic construct
  misc_feature 1..27: note = Synthetic
  source 1..27: mol_type = other DNA
caacaatattataatagtcctccactt

SEQ ID NO: 442 - protein, 9 aa, synthetic construct
  REGION 1..9: note = Synthetic
QQYYNSPPL

SEQ ID NO: 443 - DNA, 360 bp, synthetic construct
  misc_feature 1..360: note = Synthetic
  source 1..360: mol_type = other DNA
gaggtgcagctggtggagtctgggggaggcttggtacagcctggggggtccctgagactctcctgtgcagtctctggattcacctttagcaactatgccatgaactgggtccgccaggctccagggaaggggctggagtgggtctcagttattagcgacagtggtcgtagcacctactacgcagactccgtgaagggccggttcaccatctccagagacaattccaagaacacgctatatctgcaaatgaacagcctgagagccgaggacacggccgtatatttctgtgcgaaaaggtataactggaacttacactactttgactactggggccagggaaccacggtcaccgtctcctca

SEQ ID NO: 444 - protein, 120 aa, synthetic construct
  REGION 1..120: note = Synthetic
EVQLVESGGGLVQPGGSLRLSCAVSGFTFSNYAMNWVRQAPGKGLEWVSVISDSGRSTYYADSVKGRFTISRDNSKNTLYLQMNSLRAEDTAVYFCAKRYNWNLHYFDYWGQGTTVTVSS

SEQ ID NO: 445 - DNA, 24 bp, synthetic construct
  misc_feature 1..24: note = Synthetic
  source 1..24: mol_type = other DNA
ggattcacctttagcaactatgcc

SEQ ID NO: 446 - protein, 8 aa, synthetic construct
  REGION 1..8: note = Synthetic
GFTFSNYA

SEQ ID NO: 447 - DNA, 24 bp, synthetic construct
  misc_feature 1..24: note = Synthetic
  source 1..24: mol_type = other DNA
attagcgacagtggtcgtagcacc

SEQ ID NO: 448 - protein, 8 aa, synthetic construct
  REGION 1..8: note = Synthetic
ISDSGRST

SEQ ID NO: 449 - DNA, 39 bp, synthetic construct
  misc_feature 1..39: note = Synthetic
  source 1..39: mol_type = other DNA
gcgaaaaggtataactggaacttacactactttgactac

SEQ ID NO: 450 - protein, 13 aa, synthetic construct
  REGION 1..13: note = Synthetic
AKRYNWNLHYFDY

SEQ ID NO: 451 - DNA, 321 bp, synthetic construct
  misc_feature 1..321: note = Synthetic
  source 1..321: mol_type = other DNA
gaaattgtgttgacgcagtctccagactttcagtctgtgactccaaaggagaaagtcaccatcacctgccgggccagtcagagcattggtggtagcttacactggtaccagcagaaaccagatcagtctccaaagctcctcatcaagtatgcttcccagtccttctcaggggtcccctcgaggttcagtggcagtggatctgggacagatttcaccctcaccatcaatagcctggaagctgaagatgctgcaacgtattactgtcttcagagtagtagtttacggacgttcggccaagggaccaaggtggagatcaaacga

SEQ ID NO: 452 - protein, 107 aa, synthetic construct
  REGION 1..107: note = Synthetic
EIVLTQSPDFQSVTPKEKVTITCRASQSIGGSLHWYQQKPDQSPKLLIKYASQSFSGVPSRFSGSGSGTDFTLTINSLEAEDAATYYCLQSSSLRTFGQGTKVEIKR

SEQ ID NO: 453 - DNA, 18 bp, synthetic construct
  misc_feature 1..18: note = Synthetic
  source 1..18: mol_type = other DNA
cagagcattggtggtagc

SEQ ID NO: 454 - protein, 6 aa, synthetic construct
  REGION 1..6: note = Synthetic
QSIGGS

SEQ ID NO: 455-456 - skipped (2 entries)

SEQ ID NO: 457 - DNA, 24 bp, synthetic construct
  misc_feature 1..24: note = Synthetic
  source 1..24: mol_type = other DNA
cttcagagtagtagtttacggacg

SEQ ID NO: 458 - protein, 8 aa, synthetic construct
  REGION 1..8: note = Synthetic
LQSSSLRT

SEQ ID NO: 459 - DNA, 345 bp, synthetic construct
  misc_feature 1..345: note = Synthetic
  source 1..345: mol_type = other DNA
gaggtgcagctggtggagtctgggggaggcttggtacagcctggggggtccctgagactctcctgtgcagcctctggattcacctttagcagttatgccatgagctgggtccgccaggctccagggaaggggctggagtgggtctcagctattagtggtcgtggttataacgcagactacgcagactccgtgaagggccggttcaccatctccagagacaattccaagaacacgctgtatctgcaaatgaacagcctgagagccgaagacacggccgtatattactgtgcgaaattggaatactttgactactggggccagggaaccacggtcaccgtctcctca

SEQ ID NO: 460 - protein, 115 aa, synthetic construct
  REGION 1..115: note = Synthetic
EVQLVESGGGLVQPGGSLRLSCAASGFTFSSYAMSWVRQAPGKGLEWVSAISGRGYNADYADSVKGRFTISRDNSKNTLYLQMNSLRAEDTAVYYCAKLEYFDYWGQGTTVTVSS

SEQ ID NO: 461 - DNA, 24 bp, synthetic construct
  misc_feature 1..24: note = Synthetic
  source 1..24: mol_type = other DNA
ggattcacctttagcagttatgcc

SEQ ID NO: 462 - protein, 8 aa, synthetic construct
  REGION 1..8: note = Synthetic
GFTFSSYA

SEQ ID NO: 463 - DNA, 24 bp, synthetic construct
  misc_feature 1..24: note = Synthetic
  source 1..24: mol_type = other DNA
attagtggtcgtggttataacgca

SEQ ID NO: 464 - protein, 8 aa, synthetic construct
  REGION 1..8: note = Synthetic
ISGRGYNA

SEQ ID NO: 465 - DNA, 24 bp, synthetic construct
  misc_feature 1..24: note = Synthetic
  source 1..24: mol_type = other DNA
gcgaaattggaatactttgactac

SEQ ID NO: 466 - protein, 8 aa, synthetic construct
  REGION 1..8: note = Synthetic
AKLEYFDY

SEQ ID NO: 467 - DNA, 324 bp, synthetic construct
  misc_feature 1..324: note = Synthetic
  source 1..324: mol_type = other DNA
gacatccagttgacccagtctccttccaccctgtctgcatctgtaggagacagagtcaccatcacttgccgggccagtcagagtattagtagctggttggcctggtatcagcagaaaccagggaaagcccctaagctcctgatctataaggcgtctagtttagaaagtggggtcccatcaaggttcagcggcagtggatctgggacagatttcactctcaccatcagcagcctgaggcctgaagattttgcaacttattactgccaacagtataatagttaccctctgactttcggcggagggaccaaggtggaaatcaaacga

SEQ ID NO: 468 - protein, 108 aa, synthetic construct
  REGION 1..108: note = Synthetic
DIQLTQSPSTLSASVGDRVTITCRASQSISSWLAWYQQKPGKAPKLLIYKASSLESGVPSRFSGSGSGTDFTLTISSLRPEDFATYYCQQYNSYPLTFGGGTKVEIKR

SEQ ID NO: 469 - DNA, 18 bp, synthetic construct
  misc_feature 1..18: note = Synthetic
  source 1..18: mol_type = other DNA
cagagtattagtagctgg

SEQ ID NO: 470 - protein, 6 aa, synthetic construct
  REGION 1..6: note = Synthetic
QSISSW

SEQ ID NO: 471-472 - skipped (2 entries)

SEQ ID NO: 473 - DNA, 27 bp, synthetic construct
  misc_feature 1..27: note = Synthetic
  source 1..27: mol_type = other DNA
caacagtataatagttaccctctgact

SEQ ID NO: 474 - protein, 9 aa, synthetic construct
  REGION 1..9: note = Synthetic
QQYNSYPLT

SEQ ID NO: 475 - DNA, 345 bp, synthetic construct
  misc_feature 1..345: note = Synthetic
  source 1..345: mol_type = other DNA
gaggtgcagctggtggagtctgggggaggcttggtacagcctggggggtccctgagactctcctgtgcagcctctggattcacctttagcacctatgccatgcactgggtccgccaggctccagggaaggggctggagtgggtctcaagtattagtggtcgtggtcgtaactcagaccacgcagactccgtgaagggccggttcaccatctccagagacaattccaagaacacgctctatctacaaatgaacagcctgagagccgaggacacggccgtatattactgtgcgaggaccgaatacttccaccactggggccagggcaccacggtcaccgtctcctca

SEQ ID NO: 476 - protein, 115 aa, synthetic construct
  REGION 1..115: note = Synthetic
EVQLVESGGGLVQPGGSLRLSCAASGFTFSTYAMHWVRQAPGKGLEWVSSISGRGRNSDHADSVKGRFTISRDNSKNTLYLQMNSLRAEDTAVYYCARTEYFHHWGQGTTVTVSS

SEQ ID NO: 477 - DNA, 24 bp, synthetic construct
  misc_feature 1..24: note = Synthetic
  source 1..24: mol_type = other DNA
ggattcacctttagcacctatgcc

SEQ ID NO: 478 - protein, 8 aa, synthetic construct
  REGION 1..8: note = Synthetic
GFTFSTYA

SEQ ID NO: 479 - DNA, 24 bp, synthetic construct
  misc_feature 1..24: note = Synthetic
  source 1..24: mol_type = other DNA
attagtggtcgtggtcgtaactca

SEQ ID NO: 480 - protein, 8 aa, synthetic construct
  REGION 1..8: note = Synthetic
ISGRGRNS

SEQ ID NO: 481 - DNA, 24 bp, synthetic construct
  misc_feature 1..24: note = Synthetic
  source 1..24: mol_type = other DNA
gcgaggaccgaatacttccaccac

SEQ ID NO: 482 - protein, 8 aa, synthetic construct
  REGION 1..8: note = Synthetic
ARTEYFHH

SEQ ID NO: 483 - DNA, 324 bp, synthetic construct
  misc_feature 1..324: note = Synthetic
  source 1..324: mol_type = other DNA
gacatcgtgatgacccagtctccatcctcactgtctgcatctgtaggagacagaatcaccatcacttgtcgggcgagtcaggacattaacaattatttagcctggtttcagcagaaaccaggaaaagcccctaagtccctgatctatggtgcatccagcttgcaaagtggggtcccatcaaagttcagcggcagtggatctgggacagatttcactctcaccatcagcagcctgcagcctgaagattttgcaacttattactgccaacaatatacgttcttaccattcactttcggccctgggaccaaggtgaaaatcaaacga

SEQ ID NO: 484 - protein, 108 aa, synthetic construct
  REGION 1..108: note = Synthetic
DIVMTQSPSSLSASVGDRITITCRASQDINNYLAWFQQKPGKAPKSLIYGASSLQSGVPSKFSGSGSGTDFTLTISSLQPEDFATYYCQQYTFLPFTFGPGTKVKIKR

SEQ ID NO: 485 - DNA, 18 bp, synthetic construct
  misc_feature 1..18: note = Synthetic
  source 1..18: mol_type = other DNA
caggacattaacaattat

SEQ ID NO: 486 - protein, 6 aa, synthetic construct
  REGION 1..6: note = Synthetic
QDINNY

SEQ ID NO: 487-488 - skipped (2 entries)

SEQ ID NO: 489 - DNA, 27 bp, synthetic construct
  misc_feature 1..27: note = Synthetic
  source 1..27: mol_type = other DNA
caacaatatacgttcttaccattcact

SEQ ID NO: 490 - protein, 9 aa, synthetic construct
  REGION 1..9: note = Synthetic
QQYTFLPFT